European Patent Specification EP 3 941 946 B1, published December 25, 2024. Title: CLAUDIN-6 ANTIBODIES AND DRUG CONJUGATES. Applicant: THE REGENTS OF THE UNIVERSITY OF CALIFORNIA. The sequence listing filed with the application follows.

SEQUENCE LISTING (513 sequences)

SEQ ID NO: 1 - protein, 220 aa, Homo sapiens
  ref <308>: NCBI / NP_067018.2
  ref <309>: 2017-06-04
  ref <313>: (1)..(220)
MASAGMQILGVVLTLLGWVNGLVSCALPMWKVTAFIGNSIVVAQVVWEGLWMSCVVQSTGQMQCKVYDSLLALPQDLQAARALCVIALLVALFGLLVYLAGAKCTTCVEEKDSKARLVLTSGIVFVISGVLTLIPVCWTAHAIIRDFYNPLVAEAQKRELGASLYLGWAASGLLLLGGGLLCCTCPSGGSQGPSHYMARYSTSAPAISRGPSEYPTKNYV

SEQ ID NO: 2 - protein, 23 aa, Homo sapiens
WTAHAIIRDFYNPLVAEAQKREL

SEQ ID NO: 3 - protein, 13 aa, Homo sapiens
TAHAIIRDFYNPL

SEQ ID NO: 4 - protein, 10 aa, Homo sapiens
LVAEAQKREL

SEQ ID NO: 5 - protein, 220 aa, Homo sapiens
  ref <308>: NCBI / NP_001297.1
  ref <309>: 2017-07-10
  ref <313>: (1)..(220)
MSMGLEITGTALAVLGWLGTIVCCALPMWRVSAFIGSNIITSQNIWEGLWMNCVVQSTGQMQCKVYDSLLALPQDLQAARALIVVAILLAAFGLLVALVGAQCTNCVQDDTAKAKITIVAGVLFLLAALLTLVPVSWSANTIIRDFYNPVVPEAQKREMGAGLYVGWAAAALQLLGGALLCCSCPPREKKYTATKVVYSAPRSTGPGASLGTGYDRKDYV

SEQ ID NO: 6 - protein, 209 aa, Homo sapiens
  ref <308>: NCBI / NP_001296.1
  ref <309>: 2017-07-10
  ref <313>: (1)..(209)
MASMGLQVMGIALAVLGWLAVMLCCALPMWRVTAFIGSNIVTSQTIWEGLWMNCVVQSTGQMQCKVYDSLLALPQDLQAARALVIISIIVAALGVLLSVVGGKCTNCLEDESAKAKTMIVAGVVFLLAGLMVIVPVSWTAHNIIQDFYNPLVASGQKREMGASLYVGWAASGLLLLGGGLLCCNCPPRTDKPYSAKYSAARSAAASNYV

SEQ ID NO: 7 - protein, 217 aa, Homo sapiens
  ref <308>: NCBI / NP_066192.1
  ref <309>: 2017-04-15
  ref <313>: (1)..(217)
MASTGLELLGMTLAVLGWLGTLVSCALPLWKVTAFIGNSIVVAQVVWEGLWMSCVVQSTGQMQCKVYDSLLALPQDLQAARALCVIALLLALLGLLVAITGAQCTTCVEDEGAKARIVLTAGVILLLAGILVLIPVCWTAHAIIQDFYNPLVAEALKRELGASLYLGWAAAALLMLGGGLLCCTCPPPQVERPRGPRLGYSIPSRSGASGLDKRDYV

SEQ ID NO: 8 - protein, 7 aa, Artificial Sequence
  Synthetic peptide
SSVSSTY

SEQ ID NO: 9 - protein, 3 aa, Artificial Sequence
  Synthetic peptide
STS

SEQ ID NO: 10 - protein, 9 aa, Artificial Sequence
  Synthetic peptide
HQYHRSPLT

SEQ ID NO: 11 - protein, 8 aa, Artificial Sequence
  Synthetic peptide
GYTFTTYT

SEQ ID NO: 12 - protein, 8 aa, Artificial Sequence
  Synthetic peptide
INPSSGYT

SEQ ID NO: 13 - protein, 9 aa, Artificial Sequence
  Synthetic peptide
ANGDYYVAY

SEQ ID NO: 14 - protein, 6 aa, Artificial Sequence
  Synthetic peptide
ENIYSY

SEQ ID NO: 15 - protein, 3 aa, Artificial Sequence
  Synthetic peptide
NAK

SEQ ID NO: 16 - protein, 9 aa, Artificial Sequence
  Synthetic peptide
QHHYTVPWT

SEQ ID NO: 17 - protein, 8 aa, Artificial Sequence
  Synthetic peptide
GFTFSDYW

SEQ ID NO: 18 - protein, 10 aa, Artificial Sequence
  Synthetic peptide
IRLKSDNYAT

SEQ ID NO: 19 - protein, 8 aa, Artificial Sequence
  Synthetic peptide
NDGPPSGC

SEQ ID NO: 20 - protein, 6 aa, Artificial Sequence
  Synthetic peptide
ENIYSY

SEQ ID NO: 21 - protein, 3 aa, Artificial Sequence
  Synthetic peptide
NAK

SEQ ID NO: 22 - protein, 9 aa, Artificial Sequence
  Synthetic peptide
QHHYTVPWT

SEQ ID NO: 23 - protein, 8 aa, Artificial Sequence
  Synthetic peptide
GFTFSNYW

SEQ ID NO: 24 - protein, 10 aa, Artificial Sequence
  Synthetic peptide
IRLKSDNYAT

SEQ ID NO: 25 - protein, 8 aa, Artificial Sequence
  Synthetic peptide
NDGPPSGC

SEQ ID NO: 26 - protein, 11 aa, Artificial Sequence
  Synthetic peptide
QSLVHSDGNTY

SEQ ID NO: 27 - protein, 3 aa, Artificial Sequence
  Synthetic peptide
KVS

SEQ ID NO: 28 - protein, 9 aa, Artificial Sequence
  Synthetic peptide
SQSTHVPYT

SEQ ID NO: 29 - protein, 8 aa, Artificial Sequence
  Synthetic peptide
GYTFTSYT

SEQ ID NO: 30 - protein, 8 aa, Artificial Sequence
  Synthetic peptide
INPSSTYT

SEQ ID NO: 31 - protein, 10 aa, Artificial Sequence
  Synthetic peptide
SRGELGGFAY

SEQ ID NO: 32 - protein, 11 aa, Artificial Sequence
  Synthetic peptide
QSIVHSNGNTY

SEQ ID NO: 33 - protein, 3 aa, Artificial Sequence
  Synthetic peptide
KVS

SEQ ID NO: 34 - protein, 9 aa, Artificial Sequence
  Synthetic peptide
FQGSHVPFT

SEQ ID NO: 35 - protein, 8 aa, Artificial Sequence
  Synthetic peptide
GYIFTHYI

SEQ ID NO: 36 - protein, 8 aa, Artificial Sequence
  Synthetic peptide
INPYNDGT

SEQ ID NO: 37 - protein, 13 aa, Artificial Sequence
  Synthetic peptide
ARYYGYPYYSMDY

SEQ ID NO: 38 - protein, 12 aa, Artificial Sequence
  Synthetic peptide
QSLLNSRTRKNY

SEQ ID NO: 39 - protein, 3 aa, Artificial Sequence
  Synthetic peptide
WAS

SEQ ID NO: 40 - protein, 8 aa, Artificial Sequence
  Synthetic peptide
KQSYYLYT

SEQ ID NO: 41 - protein, 9 aa, Artificial Sequence
  Synthetic peptide
GYSITSGYY

SEQ ID NO: 42 - protein, 7 aa, Artificial Sequence
  Synthetic peptide
ISYDGGI

SEQ ID NO: 43 - protein, 10 aa, Artificial Sequence
  Synthetic peptide
ARFGKGAMDY

SEQ ID NO: 44 - protein, 7 aa, Artificial Sequence
  Synthetic peptide
SSVSSSY

SEQ ID NO: 45 - protein, 3 aa, Artificial Sequence
  Synthetic peptide
STS

SEQ ID NO: 46 - protein, 9 aa, Artificial Sequence
  Synthetic peptide
HQYHRSPPT

SEQ ID NO: 47 - protein, 8 aa, Artificial Sequence
  Synthetic peptide
GYSFTGYT

SEQ ID NO: 48 - protein, 8 aa, Artificial Sequence
  Synthetic peptide
INPYNGGT

SEQ ID NO: 49 - protein, 12 aa, Artificial Sequence
  Synthetic peptide
ARGVYDYDGFTY

SEQ ID NO: 50 - protein, 11 aa, Artificial Sequence
  Synthetic peptide
QSLVHSDGNTY

SEQ ID NO: 51 - protein, 3 aa, Artificial Sequence
  Synthetic peptide
KVS

SEQ ID NO: 52 - protein, 9 aa, Artificial Sequence
  Synthetic peptide
SQSTHVPYT

SEQ ID NO: 53 - protein, 8 aa, Artificial Sequence
  Synthetic peptide
GYTFTTYT

SEQ ID NO: 54 - protein, 8 aa, Artificial Sequence
  Synthetic peptide
INPRSGYS

SEQ ID NO: 55 - protein, 10 aa, Artificial Sequence
  Synthetic peptide
SRGELGGFAY

SEQ ID NO: 56 - protein, 6 aa, Artificial Sequence
  Synthetic peptide
QTIGTW

SEQ ID NO: 57 - protein, 3 aa, Artificial Sequence
  Synthetic peptide
AAA

SEQ ID NO: 58 - protein, 9 aa, Artificial Sequence
  Synthetic peptide
QQLYSIPRT

SEQ ID NO: 59 - protein, 8 aa, Artificial Sequence
  Synthetic peptide
GYRFTDYN

SEQ ID NO: 60 - protein, 8 aa, Artificial Sequence
  Synthetic peptide
INPNNGGT

SEQ ID NO: 61 - protein, 10 aa, Artificial Sequence
  Synthetic peptide
ARDYLYFFDC

SEQ ID NO: 62 - protein, 11 aa, Artificial Sequence
  Synthetic peptide
QSLVHSNGNTY

SEQ ID NO: 63 - protein, 3 aa, Artificial Sequence
  Synthetic peptide
KVS

SEQ ID NO: 64 - protein, 9 aa, Artificial Sequence
  Synthetic peptide
SQITHVPYT

SEQ ID NO: 65 - protein, 8 aa, Artificial Sequence
  Synthetic peptide
GYTFTDYS

SEQ ID NO: 66 - protein, 8 aa, Artificial Sequence
  Synthetic peptide
ISTETGEP

SEQ ID NO: 67 - protein, 10 aa, Artificial Sequence
  Synthetic peptide
TRGLWSSFAY

SEQ ID NO: 68 - protein, 10 aa, Artificial Sequence
  Synthetic peptide
KSVSTSGYSY

SEQ ID NO: 69 - protein, 3 aa, Artificial Sequence
  Synthetic peptide
LAS

SEQ ID NO: 70 - protein, 9 aa, Artificial Sequence
  Synthetic peptide
QHSRELPLT

SEQ ID NO: 71 - protein, 8 aa, Artificial Sequence
  Synthetic peptide
GFTFSSFG

SEQ ID NO: 72 - protein, 8 aa, Artificial Sequence
  Synthetic peptide
ISSDSRTI

SEQ ID NO: 73 - protein, 11 aa, Artificial Sequence
  Synthetic peptide
ARDYGRTYEAY

SEQ ID NO: 74 - protein, 6 aa, Artificial Sequence
  Synthetic peptide
QDIGGN

SEQ ID NO: 75 - protein, 3 aa, Artificial Sequence
  Synthetic peptide
STS

SEQ ID NO: 76 - protein, 9 aa, Artificial Sequence
  Synthetic peptide
LQRNAYPLT

SEQ ID NO: 77 - protein, 8 aa, Artificial Sequence
  Synthetic peptide
GFTFSSYA

SEQ ID NO: 78 - protein, 7 aa, Artificial Sequence
  Synthetic peptide
IRSGGTT

SEQ ID NO: 79 - protein, 12 aa, Artificial Sequence
  Synthetic peptide
AKVGGNPYPMDY

SEQ ID NO: 80 - protein, 7 aa, Artificial Sequence
  Synthetic peptide
SSISSNY

SEQ ID NO: 81 - protein, 3 aa, Artificial Sequence
  Synthetic peptide
RTS

SEQ ID NO: 82 - protein, 9 aa, Artificial Sequence
  Synthetic peptide
QQGSSIPLT

SEQ ID NO: 83 - protein, 8 aa, Artificial Sequence
  Synthetic peptide
GYAFSNYL

SEQ ID NO: 84 - protein, 8 aa, Artificial Sequence
  Synthetic peptide
INPGSGGT

SEQ ID NO: 85 - protein, 15 aa, Artificial Sequence
  Synthetic peptide
ARSYFGRSYPYTMDY

SEQ ID NO: 86 - protein, 10 aa, Artificial Sequence
  Synthetic peptide
QSVDYDGDNY

SEQ ID NO: 87 - protein, 3 aa, Artificial Sequence
  Synthetic peptide
AAS

SEQ ID NO: 88 - protein, 9 aa, Artificial Sequence
  Synthetic peptide
QQSNEDPFT

SEQ ID NO: 89 - protein, 8 aa, Artificial Sequence
  Synthetic peptide
GYTFTDYA

SEQ ID NO: 90 - protein, 8 aa, Artificial Sequence
  Synthetic peptide
ISTYSGNT

SEQ ID NO: 91 - protein, 13 aa, Artificial Sequence
  Synthetic peptide
ARRGDYSLYAMDY

SEQ ID NO: 92 - protein, 12 aa, Artificial Sequence
  Synthetic peptide
QSVLFSSNQKNY

SEQ ID NO: 93 - protein, 3 aa, Artificial Sequence
  Synthetic peptide
WAS

SEQ ID NO: 94 - protein, 8 aa, Artificial Sequence
  Synthetic peptide
HQYLSSRT

SEQ ID NO: 95 - protein, 8 aa, Artificial Sequence
  Synthetic peptide
GFTFSSFG

SEQ ID NO: 96 - protein, 8 aa, Artificial Sequence
  Synthetic peptide
ISSDSRTI

SEQ ID NO: 97 - protein, 11 aa, Artificial Sequence
  Synthetic peptide
ARDYGRTYEAY

SEQ ID NO: 98 - protein, 10 aa, Artificial Sequence
  Synthetic peptide
ESVDNYGISF

SEQ ID NO: 99 - protein, 3 aa, Artificial Sequence
  Synthetic peptide
AAS

SEQ ID NO: 100 - protein, 9 aa, Artificial Sequence
  Synthetic peptide
QQSKEVPLT

SEQ ID NO: 101 - protein, 8 aa, Artificial Sequence
  Synthetic peptide
GFPFSSSA

SEQ ID NO: 102 - protein, 7 aa, Artificial Sequence
  Synthetic peptide
INSDGNT

SEQ ID NO: 103 - protein, 13 aa, Artificial Sequence
  Synthetic peptide
TRNGDYRYDEFAY

SEQ ID NO: 104 - protein, 7 aa, Artificial Sequence
  Synthetic peptide
SSVSSSY

SEQ ID NO: 105 - protein, 3 aa, Artificial Sequence
  Synthetic peptide
STS

SEQ ID NO: 106 - protein, 9 aa, Artificial Sequence
  Synthetic peptide
HQYHRSPPT

SEQ ID NO: 107 - protein, 8 aa, Artificial Sequence
  Synthetic peptide
GYTFTGYW

SEQ ID NO: 108 - protein, 8 aa, Artificial Sequence
  Synthetic peptide
INPSTGYT

SEQ ID NO: 109 - protein, 12 aa, Artificial Sequence
  Synthetic peptide
AREGITTVLVDY

SEQ ID NO: 110 - protein, 12 aa, Artificial Sequence
  Synthetic peptide
QSVLFSSNQKNY

SEQ ID NO: 111 - protein, 3 aa, Artificial Sequence
  Synthetic peptide
WAS

SEQ ID NO: 112 - protein, 8 aa, Artificial Sequence
  Synthetic peptide
HQYLSSRT

SEQ ID NO: 113 - protein, 8 aa, Artificial Sequence
  Synthetic peptide
GYSFTGYN

SEQ ID NO: 114 - protein, 8 aa, Artificial Sequence
  Synthetic peptide
IDPYYGGS

SEQ ID NO: 115 - protein, 14 aa, Artificial Sequence
  Synthetic peptide
ARERSGYVFSAMDY

SEQ ID NO: 116 - protein, 12 aa, Artificial Sequence
  Synthetic peptide
QSVLFSSNQKNY

SEQ ID NO: 117 - protein, 3 aa, Artificial Sequence
  Synthetic peptide
WAS

SEQ ID NO: 118 - protein, 8 aa, Artificial Sequence
  Synthetic peptide
HQYLSSRT

SEQ ID NO: 119 - protein, 8 aa, Artificial Sequence
  Synthetic peptide
GYSFTGYT

SEQ ID NO: 120 - protein, 8 aa, Artificial Sequence
  Synthetic peptide
INPYNGVT

SEQ ID NO: 121 - protein, 16 aa, Artificial Sequence
  Synthetic peptide
TRDPLYYGYRDSTMDY

SEQ ID NO: 122 - protein, 11 aa, Artificial Sequence
  Synthetic peptide
QSLVHSDGNTY

SEQ ID NO: 123 - protein, 3 aa, Artificial Sequence
  Synthetic peptide
KVS

SEQ ID NO: 124 - protein, 9 aa, Artificial Sequence
  Synthetic peptide
SQSTHVPYT

SEQ ID NO: 125 - protein, 8 aa, Artificial Sequence
  Synthetic peptide
GYTFTSYT

SEQ ID NO: 126 - protein, 8 aa, Artificial Sequence
  Synthetic peptide
INPSSTYT

SEQ ID NO: 127 - protein, 10 aa, Artificial Sequence
  Synthetic peptide
SRGELGGFAY

SEQ ID NO: 128 - protein, 6 aa, Artificial Sequence
  Synthetic peptide
QGIRGN

SEQ ID NO: 129 - protein, 3 aa, Artificial Sequence
  Synthetic peptide
STS

SEQ ID NO: 130 - protein, 9 aa, Artificial Sequence
  Synthetic peptide
LQRNAYPLT

SEQ ID NO: 131 - protein, 8 aa, Artificial Sequence
  Synthetic peptide
GFTFSSFA

SEQ ID NO: 132 - protein, 7 aa, Artificial Sequence
  Synthetic peptide
IRSGGIT

SEQ ID NO: 133 - protein, 13 aa, Artificial Sequence
  Synthetic peptide
ARVSTATYYGMDY

SEQ ID NO: 134 - protein, 108 aa, Artificial Sequence
  Synthetic peptide
QIVLTQSPAIMSASLGERVTMTCTASSSVSSTYFHWYQQKPGSSPKLWIYSTSNLASGVPRRFSGSASGTSYSLTISSMEAEDAATYYCHQYHRSPLTFGAGTKLELK

SEQ ID NO: 135 - protein, 116 aa, Artificial Sequence
  Synthetic peptide
QVQLQQSAAELARPGASVKMSCKASGYTFTTYTMHWVKQRPGQGLEWIGFINPSSGYTDYNQKFKDRTTLTADKSSSTVYMQLSSLTSEDSAVYYCANGDYYVAYWGQGTLVTVSA

SEQ ID NO: 136 - protein, 107 aa, Artificial Sequence
  Synthetic peptide
DIQMTQSPASLSASVGETVTITCRISENIYSYLAWYQQKQGKSPQLLVYNAKILVEGVPSRFSGSGSGTQFSLKINSLQPEDFGNYYCQHHYTVPWTFGGGTKLEIK

SEQ ID NO: 137 - protein, 117 aa, Artificial Sequence
  Synthetic peptide
EVKLEESGGGLVQPGGSMKLSCVASGFTFSDYWMNWVRQSPEKGLEWVAQIRLKSDNYATHYAESVKGRFTISRDDSKRSVYLQMNNLRAEDTGTYYCNDGPPSGCWGQGTTLIVSS

SEQ ID NO: 138 - protein, 107 aa, Artificial Sequence; identical to SEQ ID NO: 136
  Synthetic peptide

SEQ ID NO: 139 - protein, 117 aa, Artificial Sequence
  Synthetic peptide
EVKLEESGGGLVQPGGSMKLSCVASGFTFSNYWMNWVRQSPEKGLEWVAQIRLKSDNYATHYAESVKGRFTISRDDSKRSVYLQMNNLRAEDTGTYYCNDGPPSGCWGQGTTLIVSS

SEQ ID NO: 140 - protein, 112 aa, Artificial Sequence
  Synthetic peptide
DVVMTQTPLSLPVSLGDQASISCRSSQSLVHSDGNTYLNWYLQKPGQSPKLLIYKVSNRFSGVPDRFSGSGSGTDFTLKIRRVEAEDLGVYFCSQSTHVPYTFGGGTKLEIK

SEQ ID NO: 141 - protein, 117 aa, Artificial Sequence
  Synthetic peptide
QVQLQQSGAELARPGASVKMSCKASGYTFTSYTMHWIKQRPGQGQEWIGYINPSSTYTHYIKKFKDKATLTADKSSSTAYMQLRSLTSEDSAVYYCSRGELGGFAYWGQGTLVTVSA

SEQ ID NO: 142 - protein, 112 aa, Artificial Sequence
  Synthetic peptide
DVLMTQTPLSLPVSLGDQPSISCRSSQSIVHSNGNTYLDWYLQKPGQSPKLLIYKVSNRFSGVPDRFSGSGSGTDFTLKISRVEAEDLGVYYCFQGSHVPFTFGSGTRLEIK

SEQ ID NO: 143 - protein, 120 aa, Artificial Sequence
  Synthetic peptide
EVQLQQSGPELVKPGASVKMSCKASGYIFTHYIMHWVKQKPGQGLEWIGCINPYNDGTKYNEKFKGKATLTSDKSSSTAYMELSSLTSEDSAVYYCARYYGYPYYSMDYWGQGTSVTVSS

SEQ ID NO: 144 - protein, 112 aa, Artificial Sequence
  Synthetic peptide
AIVMFQSPSSLVVSAGEKVTMSCKSSQSLLNSRTRKNYLAWYQQKPGQSPKLLIYWASTRESGVPDRFTGSGSGTDFTLTISSVQAEDLAVYYCKQSYYLYTFGGGTKLEIK

SEQ ID NO: 145 - protein, 117 aa, Artificial Sequence
  Synthetic peptide
DVQLQESGPGLVKSSQSLSLTCSVTGYSITSGYYWKWIRQFPGNKLEWMGYISYDGGINYNPSLKNRISITRDTSKNQFFLKLNSVTTEDTAKYYCARFGKGAMDYWGQGTSVTVSS

SEQ ID NO: 146 - protein, 108 aa, Artificial Sequence
  Synthetic peptide
QIVLTQSPAIMSASLGDRVTMTCTASSSVSSSYLHWYQQKPGSSPKLWIYSTSNLASGVPARFSGSGSGTSYSLTISSMEAEDAATYYCHQYHRSPPTFGSGTKLEIK

SEQ ID NO: 147 - protein, 119 aa, Artificial Sequence
  Synthetic peptide
EVQLQQSGPELVKPGASMKISCKASGYSFTGYTMNWVKQSHGKNLEWIGLINPYNGGTNYNQKFKGKATLTVDKSSSTAYMELLSLTSEDSAVYYCARGVYDYDGFTYWGQGTLVTVSA

SEQ ID NO: 148 - protein, 112 aa, Artificial Sequence
  Synthetic peptide
DVVMTQTPLSLPVSLGDQASISCRSSQSLVHSDGNTYLYWYLQKPGQSPKLLIYKVSNRFSGVPDRFSGSGSGTDFTLKISRVEAEDLGVYFCSQSTHVPYTFGGGTKLEIK

SEQ ID NO: 149 - protein, 117 aa, Artificial Sequence
  Synthetic peptide
QVQLQQSGAELARPGASVKMSCKASGYTFTTYTMHWLKQRPGQGLEWIGYINPRSGYSNYNQKFKDKATLTADKSSNTAYMQLNTLTSEDSKVYYCSRGELGGFAYWGQGTLVTVSA

SEQ ID NO: 150 - protein, 107 aa, Artificial Sequence
  Synthetic peptide
DIQMTQSPASQSASLGESVTITCLASQTIGTWLAWYQQKPGKSPQLLIYAAASLADGVPSRFSGSGSGTRFSFKISSLQAEDFVSYYCQQLYSIPRTFGGGTKLEIK

SEQ ID NO: 151 - protein, 117 aa, Artificial Sequence
  Synthetic peptide
EVQLQQSGPELVKPGASVKMSCKASGYRFTDYNMHWVKQSHGKSLEWIGYINPNNGGTNYNQNFKGKATLTVNKSSSTAYMELRSLTSEDSAAYYCARDYLYFFDCWGQGTTLTVSS

SEQ ID NO: 152 - protein, 112 aa, Artificial Sequence
  Synthetic peptide
DVVMTQTPLSLPVSLGDQASISCRASQSLVHSNGNTYLHWFLQKPGQSPKLLIYKVSNRFSGVPDRFSGSGSRTDFTLKISRVEAEDLGVYFCSQITHVPYTFGGGTKLEIK

SEQ ID NO: 153 - protein, 117 aa, Artificial Sequence
  Synthetic peptide
QIQLVQSGPALKKPGETVKISCKASGYTFTDYSMHWIKQAPGKGLKWMGWISTETGEPTYADGFKGRFDFSLETSADTAYLSINNLTNEDTATYFCTRGLWSSFAYWGQGTLVTVSA

SEQ ID NO: 154 - protein, 111 aa, Artificial Sequence
  Synthetic peptide
DIVLTQSPASLAVSLGQRATISCRASKSVSTSGYSYIHWYQQKPGQPPKLLIYLASNLESGVPARFSGSGSGTDFTLNIHPVEEEDAATYYCQHSRELPLTFGAGTKLELK

SEQ ID NO: 155 - protein, 118 aa, Artificial Sequence
  Synthetic peptide
DVQLVESGGGLVQPRGSRKLSCAASGFTFSSFGMHWVRQAPEKGLEWVAYISSDSRTIYYADTVKGRFTISRDNPTNTLFLQMTSLRSEDTAMYYCARDYGRTYEAYWGQGTLVTVSA

SEQ ID NO: 156 - protein, 107 aa, Artificial Sequence
  Synthetic peptide
DIQMIQSPSSMFASLGDRVSLSCRASQDIGGNLDWYQQKPGGTIKLLIYSTSNLNSGVPSRFSGSGSGSDYSLTITSLESEDFADYYCLQRNAYPLTFGAGTKLELK

SEQ ID NO: 157 - protein, 118 aa, Artificial Sequence
  Synthetic peptide
EVKLMESGGDLVKPGGSLKLSCAASGFTFSSYAMSWVRQTPEKRLEWVASIRSGGTTYYPDSVKGRFTISRDNARNILYLRMSSLRSEDTAIYYCAKVGGNPYPMDYWGQGTSVTVSS

SEQ ID NO: 158 - protein, 108 aa, Artificial Sequence
  Synthetic peptide
EIVLTQSPTTMAASPGEKITITCSASSSISSNYLHWYQQKPGFSPKLLIYRTSNLASGVPARFSGSGSGTSYSLTIGTMEAEDVATYYCQQGSSIPLTFGAGTKLELK

SEQ ID NO: 159 - protein, 122 aa, Artificial Sequence
  Synthetic peptide
QVQLQQSGAELVRPGTSVKVSCKASGYAFSNYLIEWVKQRPGQGLEWIGVINPGSGGTNYNEKFKGKATMTADKSSSTAYMHLSNLTSEDSVVYFCARSYFGRSYPYTMDYWGQGTSVTVSS

SEQ ID NO: 160 - protein, 111 aa, Artificial Sequence
  Synthetic peptide
DIVLTQSPASLAVSLGQRATISCKASQSVDYDGDNYVNWYQQKVGQPPKLLISAASNLESGIPARFSGSGSGTDFTLNIHPVEEEDAATYYCQQSNEDPFTFGSGTKLEIK

SEQ ID NO: 161 - protein, 120 aa, Artificial Sequence
  Synthetic peptide
QVQLQQSGPELVRPGVSVKISCKGSGYTFTDYAMHWVKQSHAKSLEWIGVISTYSGNTNYNQKFQDKATMTVDKSSSTAYMALARLTSDDSAIYYCARRGDYSLYAMDYWGQGTSVTVSS

SEQ ID NO: 162 - protein, 112 aa, Artificial Sequence
  Synthetic peptide
NIMMTQSPSSLAVSAGEKVTMSCKSSQSVLFSSNQKNYLAWYQQKPGQSPRLLIYWASTRESGVPDRFTGSGSGTDFTLTISNVQAEDLAVYYCHQYLSSRTFGAGTKLELK

SEQ ID NO: 163 - protein, 118 aa, Artificial Sequence; identical to SEQ ID NO: 155
  Synthetic peptide

SEQ ID NO: 164 - protein, 111 aa, Artificial Sequence
  Synthetic peptide
DIVLTQSPASLALSLGQRATISCRASESVDNYGISFMNWFQQKPGQPPKLLIYAASNQGSGVPARFSGSGSGTDFSLNIHPMEEDDTAMYFCQQSKEVPLTFGAGTKLELK

SEQ ID NO: 165 - protein, 119 aa, Artificial Sequence
  Synthetic peptide
EVRLVESGGGLMQPGGSLKLPCAASGFPFSSSAMSWVRQTPEKRLEWVASINSDGNTYYPDSVKGRFTISRDSARNILYLQMSSLRSEDTAMYYCTRNGDYRYDEFAYWGQGTLVTVSA

SEQ ID NO: 166 - protein, 108 aa, Artificial Sequence
  Synthetic peptide
QIVLTQSPAIMSASLGERVTMTCTASSSVSSSYLHWYQQKPGSSPKLWIYSTSNLASGVPARFSGSGSGTSYSLTISSMEAEDAATYYCHQYHRSPPTFGAGTKLELK

SEQ ID NO: 167 - protein, 119 aa, Artificial Sequence
  Synthetic peptide
QVQLQQSGAELAKPGASVKMSCKASGYTFTGYWMHWVKQRPGQGLEWLGYINPSTGYTESNQKFKDKATLTADKSSTTAYMQLRSLTPEDSAVYYCAREGITTVLVDYWGQGTTLTVSS

SEQ ID NO: 168 - protein, 112 aa, Artificial Sequence; identical to SEQ ID NO: 162
  Synthetic peptide

SEQ ID NO: 169 - protein, 121 aa, Artificial Sequence
  Synthetic peptide
QVQLKQSGPELEKPGASVKISCKASGYSFTGYNMNWVKQSNGKSLEWIGNIDPYYGGSTYNQKFTGKATLTVDKSSSTAYMQLKSLTSEDSAVYYCARERSGYVFSAMDYWGQGTSVTVSS

SEQ ID NO: 170 - protein, 112 aa, Artificial Sequence; identical to SEQ ID NO: 162
  Synthetic peptide

SEQ ID NO: 171 - protein, 123 aa, Artificial Sequence
  Synthetic peptide
EVQLQQSGPELVKPGGSMKISCKASGYSFTGYTMNWVKRSHGKNLEWIGLINPYNGVTTYNQNFKGKATLAVDKSSSTAYMELLGLTSEDSAVYYCTRDPLYYGYRDSTMDYWGQGTSVTVSS

SEQ ID NO: 172 - protein, 112 aa, Artificial Sequence; identical to SEQ ID NO: 140
  Synthetic peptide

SEQ ID NO: 173 - protein, 117 aa, Artificial Sequence
  Synthetic peptide
EVQLQQSGAELARPGASVKMSCKASGYTFTSYTMHWIKQRPGQGQEWIGYINPSSTYTHYIKKFKDKATLTADKSSSTAYMQLRSLTSEDSAVYYCSRGELGGFAYWGQGTLVTVSA

SEQ ID NO: 174 - protein, 107 aa, Artificial Sequence
  Synthetic peptide
DIQMIQSPSSMFASLGDRVSLSCRASQGIRGNLDWYQQKPGGTIKLLIYSTSILNSGVPSRFSGSGSGSDYSLTITSLESEDFADYYCLQRNAYPLTFGSGTKLELK

SEQ ID NO: 175 - protein, 119 aa, Artificial Sequence
  Synthetic peptide
EVKLVESGGGLMKPGGSLKLSCAASGFTFSSFALSWVRQTPEKRLEWVASIRSGGITYHADSVKGRFTISRDNAGNILYLQMNSLRSEDTAMYFCARVSTATYYGMDYWGQGTSVTVSS

SEQ ID NO: 176 - protein, 219 aa, Mus musculus
  ref <308>: NCBI / NP_061247.1
  ref <309>: 2017-08-07
  ref <313>: (1)..(219)
MASTGLQILGIVLTLLGWVNALVSCALPMWKVTAFIGNSIVVAQMVWEGLWMSCVVQSTGQMQCKVYDSLLALPQDLQAARALCVVTLLIVLLGLLVYLAGAKCTTCVEDRNSKSRLVLISGIIFVISGVLTLIPVCWTAHSIIQDFYNPLVADAQKRELGASLYLGWAASGLLLLGGGLLCCACSSGGTQGPRHYMACYSTSVPHSRGPSEYPTKNYV

SEQ ID NO: 177 - protein, 80 aa, Artificial Sequence
  Synthetic peptide
MASAGMQILGVVLTLLGWVNGLVSCALPMWKVTAFIGNSIVVAQVVWEGLWMSCVVQSTGQMQCKVYDSLLALPQDLQAA

SEQ ID NO: 178 - protein, 220 aa, Artificial Sequence
  Synthetic peptide
MASAGMQILGVVLTLLGWVNGLVSCALPMWKVTAFIGNSIVVAQVVWEGLWMSCVVQSTGQMQCKVYDSLLALPQDLQAARALCVIALLVALFGLLVYLAGAKCTTCVEEKDSKARLVLTSGIVFVISGVLTLIPVCWTAHAVIRDFYNPLVAEAQKRELGASLYLGWAASGLLLLGGGLLCCTCPSGGSQGPSHYMARYSTSAPAISRGPSEYPTKNYV

SEQ ID NO: 179 - protein, 322 aa, Artificial Sequence
  Synthetic peptide
CAGATCGTGCTGACTCAGAGTCCTTCAATTATGTCCGTGAGCCCAGGCGAGAAGGTCACCATCACATGCAGTGCCTCCAGCTCTGTCTCATACATGCACTGGTTCCAGCAGAAGCCAGGGACCAGTCCCAAGCTGTGCATCTACTCTACATCGAACCTGGCCTCCGGAGTGCCCGCAAGGTTTAGCGGTCGGGGCTCTGGAACTTCATACTCCCTGACCATCTCGCGGGTGGCCGCTGAGGATGCAGCAACATACTATTGCCAGCAGAGGTCCAATTATCCCCCTTGGACATTCGGCGGAGGTACCAAACTCGAGATTAAGC

SEQ ID NO: 180 - protein, 351 aa, Artificial Sequence
  Synthetic peptide
GAAGTCCAGCTGCAGCAGTCTGGCCCTGAACTGGTGAAGCCTGGCGCCAGCATGAAGATCTCCTGCAAGGCCAGCGGCTACTCCTTCACCGGCTATACAATGAACTGGGTGAAGCAGTCCCACGGCAAGAATCTGGAGTGGATCGGCCTGATCAACCCATACAATGGCGGCACCATCTACAACCAGAAGTTTAAGGGCAAGGCCACCCTGACAGTGGACAAGAGCTCCTCTACCGCCTACATGGAGCTGCTGTCTCTGACAAGCGAGGACTCCGCCGTGTACTATTGCGCCCGGGACTACGGCTTCGTGCTGGACTATTGGGGCCAGGGCACCACACTGACAGTGAGCTCC

SEQ ID NO: 181 - protein, 107 aa, Artificial Sequence
  Synthetic peptide
QIVLTQSPSIMSVSPGEKVTITCSASSSVSYMHWFQQKPGTSPKLCIYSTSNLASGVPARFSGRGSGTSYSLTISRVAAEDAATYYCQQRSNYPPWTFGGGTKLEIK

SEQ ID NO: 182 - protein, 117 aa, Artificial Sequence
  Synthetic peptide
EVQLQQSGPELVKPGASMKISCKASGYSFTGYTMNWVKQSHGKNLEWIGLINPYNGGTIYNQKFKGKATLTVDKSSSTAYMELLSLTSEDSAVYYCARDYGFVLDYWGQGTTLTVSS

SEQ ID NO: 183 - DNA, 324 bp, Artificial Sequence
  Synthetic polynucleotide
gaaattgtgctcacccagtctccagcactcatggctgcatctccaggggagaaggtcaccatcacctgcagtgtcagctcaagtataagttccagcaacttgcactggtaccagcagaagtcaggaacctcccccaaactctggatttatggcacatccaacctggcttctggagtccctgttcgcttcagtggcagtggatctgggacctcttattctctcacaatcagcaacatggaggctgaagatgctgccacttattactgtcaacagtggagtagttacccacacacgttcggaggggggaccaagctggaaataaaa

SEQ ID NO: 184 - DNA, 378 bp, Artificial Sequence
  Synthetic polynucleotide
caggtccaaatgcagcagtctggagctgagctggtaaggcctgggacttcagtgaaggtgtcctgcaaggcttctggatacgccttcactaattacttgatagagtgggtaaagcagaggcctggacagggccttgagtggattggactgattaatcctggaagtggtggtactaattacaatgagaagttcaagggcaaggcaacactgactgcagacaaatcctccaccactgcctacatgcagctcagcagcctgacatctgatgactctgcggtttatttctgtgcaagacggtcccctctagggagttggatctactatgcttacgacggtgttgcttactggggccaagggactctggtcactgtctctgca

SEQ ID NO: 185 - protein, 108 aa, Artificial Sequence
  Synthetic peptide
EIVLTQSPALMAASPGEKVTITCSVSSSISSSNLHWYQQKSGTSPKLWIYGTSNLASGVPVRFSGSGSGTSYSLTISNMEAEDAATYYCQQWSSYPHTFGGGTKLEIK

SEQ ID NO: 186 - protein, 126 aa, Artificial Sequence
  Synthetic peptide
QVQMQQSGAELVRPGTSVKVSCKASGYAFTNYLIEWVKQRPGQGLEWIGLINPGSGGTNYNEKFKGKATLTADKSSTTAYMQLSSLTSDDSAVYFCARRSPLGSWIYYAYDGVAYWGQGTLVTVSA

SEQ ID NO: 187 - DNA, 645 bp, Mus musculus
gatattgtgctaactcagtctccagccaccctgtctgtgactccaggaaatagcgtcagtctttcctgcagggccagccaaagtattggcggtaacctacactggtatcaacaaaaatcacatgagtctccaaggcttctcatcaagtatgcttcccagtccatctctgggatcccctccaggttcagtggcagtggatcagggacagatttcactctcagtatcaacagtgtggagactgaagattttggaatgtatttctgtcaacagagtaacagctggccttacacgttcggaggggggaccaagctggaaataaaacgggcagatgctgcaccaactgtatccatcttcccaccatccagtgagcagttaacatctggaggtgcctcagtcgtgtgcttcttgaacaacttctaccccaaagacatcaatgtcaagtggaagattgatggcagtgaacgacaaaatggcgtcctgaacagttggactgatcaggacagcaaagacagcacctacagcatgagcagcaccctcacgttgaccaaggacgagtatgaacgacataacagctatacctgtgaggccactcacaagacatcaacttcacccattgtcaagagcttcaacaggaatgagtgttag

SEQ ID NO: 188 - DNA, 1335 bp, Mus musculus
gacgtgcagcttcaggagtcaggacctagcctcgtgaaaccttctcagactctgtccctcacctgttctgtcactggcgactccatcaccagtgattactggagctggatccggaaattcccagggaatagacttgagtacatggggtacgtaagctacagtggtagcacttactacaatccatctctcaaaagtcgaatctccatcacccgagacacatccaagaaccagtactacctggatttgaattctgtgactactgaggacacagccacatattactgtgcaaactgggacggtgattactggggccaagggactctggtcactgtctcttcagcagctaaaacaacagccccatcggtctatccactggcccctgtgtgtggagatacaactggctcctcggtgactctaggatgcctggtcaagggttatttccctgagccagtgaccttgacctggaactctggatccctgtccagtggtgtgcacaccttcccagctgtcctgcagtctgacctctacaccctcagcagctcagtgactgtaacctcgagcacctggcccagccagtccatcacctgcaatgtggcccacccggcaagcagcaccaaggtggacaagaaaattgagcccagagggcccacaatcaagccctgtcctccatgcaaatgcccagcacctaacctcttgggtggaccatccgtcttcatcttccctccaaagatcaaggatgtactcatgatctccctgagccccatagtcacatgtgtggtggtggatgtgagcgaggatgacccagatgtccagatcagctggtttgtgaacaacgtggaagtacacacagctcagacacaaacccatagagaggattacaacagtactctccgggtggtcagtgccctccccatccagcaccaggactggatgagtggcaaggagttcaaatgcaaggtcaacaacaaagacctcccagcgcccatcgagagaaccatctcaaaacccaaagggtcagtaagagctccacaggtatatgtcttgcctccaccagaagaagagatgactaagaaacaggtcactctgacctgcatggtcacagacttcatgcctgaagacatttacgtggagtggaccaacaacgggaaaacagagctaaactacaagaacactgaaccagtcctggactctgatggttcttacttcatgtacagcaagctgagagtggaaaagaagaactgggtggaaagaaatagctactcctgttcagtggtccacgagggtctgcacaatcaccacacgactaagagcttctcccggactccgggtaaatga

SEQ ID NO: 189 - DNA, 8806 bp, Artificial Sequence
  Synthetic peptide
aatgtagtcttatgcaatactcttgtagtcttgcaacatggtaacgatgagttagcaacatgccttacaaggagagaaaaagcaccgtgcatgccgattggtggaagtaaggtggtacgatcgtgccttattaggaaggcaacagacgggtctgacatggattggacgaaccactgaattgccgcattgcagagatattgtatttaagtgcctagctcgatacataaacgggtctctctggttagaccagatctgagcctgggagctctctggctaactagggaacccactgcttaagcctcaataaagcttgccttgagtgcttcaagtagtgtgtgcccgtctgttgtgtgactctggtaactagagatccctcagacccttttagtcagtgtggaaaatctctagcagtggcgcccgaacagggacttgaaagcgaaagggaaaccagaggagctctctcgacgcaggactcggcttgctgaagcgcgcacggcaagaggcgaggggcggcgactggtgagtacgccaaaaattttgactagcggaggctagaaggagagagatgggtgcgagagcgtcagtattaagcgggggagaattagatcgcgatgggaaaaaattcggttaaggccagggggaaagaaaaaatataaattaaaacatatagtatgggcaagcagggagctagaacgattcgcagttaatcctggcctgttagaaacatcagaaggctgtagacaaatactgggacagctacaaccatcccttcagacaggatcagaagaacttagatcattatataatacagtagcaaccctctattgtgtgcatcaaaggatagagataaaagacaccaaggaagctttagacaagatagaggaagagcaaaacaaaagtaagaccaccgcacagcaagcggccgctgatcttcagacctggaggaggagatatgagggacaattggagaagtgaattatataaatataaagtagtaaaaattgaaccattaggagtagcacccaccaaggcaaagagaagagtggtgcagagagaaaaaagagcagtgggaataggagctttgttccttgggttcttgggagcagcaggaagcactatgggcgcagcgtcaatgacgctgacggtacaggccagacaattattgtctggtatagtgcagcagcagaacaatttgctgagggctattgaggcgcaacagcatctgttgcaactcacagtctggggcatcaagcagctccaggcaagaatcctggctgtggaaagatacctaaaggatcaacagctcctggggatttggggttgctctggaaaactcatttgcaccactgctgtgccttggaatgctagttggagtaataaatctctggaacagatttggaatcacacgacctggatggagtgggacagagaaattaacaattacacaagcttaatacactccttaattgaagaatcgcaaaaccagcaagaaaagaatgaacaagaattattggaattagataaatgggcaagtttgtggaattggtttaacataacaaattggctgtggtatataaaattattcataatgatagtaggaggcttggtaggtttaagaatagtttttgctgtactttctatagtgaatagagttaggcagggatattcaccattatcgtttcagacccacctcccaaccccgaggggacccgacaggcccgaaggaatagaagaagaaggtggagagagagacagagacagatccattcgattagtgaacggatctcgacggtatcggttaacttttaaaagaaaaggggggattggggggtacagtgcaggggaaagaatagtagacataatagcaacagacatacaaactaaagaattacaaaaacaaattacaaaaattcaaaattttccgataagcttgggagttccgcgttacataacttacggtaaatggcccgcctggctgaccgcccaacgacccccgcccattgacgtcaataatgacgtatgttcccatagtaacgccaatagggactttccattgacgtcaatgggtggagtatttacggtaaactgcccacttggcagtacatcaagtgtatcatatgccaagtacgccccctattgacgtcaatgacggtaaatggcccgcctggcattatgcccagtacatgaccttatgggactttcctacttggcagtacatctacgtattagtcatcgctattaccatggtgatgcggttttggcagtacatcaatgggcgtggatagcggtttgactcacggggatttccaagtctccaccccattgacgtcaatgggagtttgttttggcaccaaaatcaacgggactttccaaaatgtcgtaacaactccgccccattgacgcaaatgggcggtaggcgtgtacggtgggaggtctatataagcagagctcgtttagtgaaccgtcagatcgcctggagacgccatccacgctgttttgacctccatagaagacaccgactctagaactagtggatcccccgggctgcaggaattcgtcgactggatccggtaccgaggagatctgccgccgcgatcgccggcgcgccagatctcaagcttaactagttagcggaccgacgcgtacgcggccgctcgagatgagcgggggcgaggagctgttcgccggcatcgtgcccgtgctgatcgagctggacggcgacgtgcacggccacaagttcagcgtgcgcggcgagggcgagggcgacgccgactacggcaagctggagatcaagttcatctgcaccaccggcaagctgcccgtgccctggcccaccctggtgaccaccctctgctacggcatccagtgcttcgcccgctaccccgagcacatgaagatgaacgacttcttcaagagcgccatgcccgagggctacatccaggagcgcaccatccagttccaggacgacggcaagtacaagacccgcggcgaggtgaagttcgagggcgacaccctggtgaaccgcatcgagctgaagggcaaggacttcaaggaggacggcaacatcctgggccacaagctggagtacagcttcaacagccacaacgtgtacatccgccccgacaaggccaacaacggcctggaggctaacttcaagacccgccacaacatcgagggcggcggcgtgcagctggccgaccactaccagaccaacgtgcccctgggcgacggccccgtgctgatccccatcaaccactacctgagcactcagaccaagatcagcaaggaccgcaacgaggcccgcgaccacatggtgctcctggagtccttcagcgcctgctgccacacccacggcatggacgagctgtacaggtccggactcagataagtttaaacccgatatcatcatctagggcggccaattccgcccctctccccccccctaacgttactggccgaagccgcttggaataaggccggtgtgcgtttgtctatatgttattttccaccatattgccgtcttttggcaatgtgagggcccggaaacctggccctgtcttcttgacgagcattcctaggggtctttcccctctcgccaaaggaatgcaaggtctgttgaatgtcgtgaaggaagcagttcctctggaagcttcttgaagacaaacaacgtctgtagcgaccctttgcaggcagcggaaccccccacctggcgacaggtgcctctgcggccaaaagccacgtgtataagatacacctgcaaaggcggcacaaccccagtgccacgttgtgagttggatagttgtggaaagagtcaaatggctctcctcaagcgtattcaacaaggggctgaaggatgcccagaaggtaccccattgtatgggatctgatctggggcctcggtgcacatgctttacatgtgtttagtcgaggttaaaaaaacgtctaggccccccgaaccacggggacgtggttttcctttgaaaaacacgatgataagcttgccacaacccacaaggagacgaccttccatgaccgagtacaagcccacggtgcgcctcgccacccgcgacgacgtcccccgggccgtacgcaccctcgccgccgcgttcgccgactaccccgccacgcgccacaccgtcgacccggaccgccacatcgagcgggtcaccgagctgcaagaactcttcctcacgcgcgtcgggctcgacatcggcaaggtgtgggtcgcggacgacggcgccgcggtggcggtctggaccacgccggagagcgtcgaagcgggggcggtgttcgccgagatcggcccgcgcatggccgagttgagcggttcccggctggccgcgcagcaacagatggaaggcctcctggcgccgcaccggcccaaggagcccgcgtggttcctggccaccgtcggcgtctcgcccgaccaccagggcaagggtctgggcagcgccgtcgtgctccccggagtggaggcggccgagcgcgccggggtgcccgccttcctggagacctccgcgccccgcaacctccccttctacgagcggctcggcttcaccgtcaccgccgacgtcgaggtgcccgaaggaccgcgcacctggtgcatgacccgcaagcccggtgcctgaaattagatcgataccgtcgacaatcaacctctggattacaaaatttgtgaaagattgactggtattcttaactatgttgctccttttacgctatgtggatacgctgctttaatgcctttgtatcatgctattgcttcccgtatggctttcattttctcctccttgtataaatcctggttgctgtctctttatgaggagttgtggcccgttgtcaggcaacgtggcgtggtgtgcactgtgtttgctgacgcaacccccactggttggggcattgccaccacctgtcagctcctttccgggactttcgctttccccctccctattgccacggcggaactcatcgccgcctgccttgcccgctgctggacaggggctcggctgttgggcactgacaattccgtggtgttgtcggggaagctgacgtcctttccatggctgctcgcctgtgttgccacctggattctgcgcgggacgtccttctgctacgtcccttcggccctcaatccagcggaccttccttcccgcggcctgctgccggctctgcggcctcttccgcgtcttcgccttcgccctcagacgagtcggatctccctttgggccgcctccccgcctgaatacgagctcggtacctttaagaccaatgacttacaaggcagctgtagatcttagccactttttaaaagaaaaggggggactggaagggctaattcactcccaacgaagacaagatctgctttttgcttgtactgggtctctctggttagaccagatctgagcctgggagctctctggctaactagggaacccactgcttaagcctcaataaagcttgccttgagtgcttcaagtagtgtgtgcccgtctgttgtgtgactctggtaactagagatccctcagacccttttagtcagtgtggaaaatctctagcagtagtagttcatgtcatcttattattcagtatttataacttgcaaagaaatgaatatcagagagtgagaggaacttgtttattgcagcttataatggttacaaataaagcaatagcatcacaaatttcacaaataaagcatttttttcactgcattctagttgtggtttgtccaaactcatcaatgtatcttatcatgtctggctctagctatcccgcccctaactccgcccatcccgcccctaactccgcccagttccgcccattctccgccccatggctgactaattttttttatttatgcagaggccgaggccgcctcggcctctgagctattccagaagtagtgaggaggcttttttggaggcctagggacgtacccaattcgccctatagtgagtcgtattacgcgcgctcactggccgtcgttttacaacgtcgtgactgggaaaaccctggcgttacccaacttaatcgccttgcagcacatccccctttcgccagctggcgtaatagcgaagaggcccgcaccgatcgcccttcccaacagttgcgcagcctgaatggcgaatgggacgcgccctgtagcggcgcattaagcgcggcgggtgtggtggttacgcgcagcgtgaccgctacacttgccagcgccctagcgcccgctcctttcgctttcttcccttcctttctcgccacgttcgccggctttccccgtcaagctctaaatcgggggctccctttagggttccgatttagtgctttacggcacctcgaccccaaaaaacttgattagggtgatggttcacgtagtgggccatcgccctgatagacggtttttcgccctttgacgttggagtccacgttctttaatagtggactcttgttccaaactggaacaacactcaaccctatctcggtctattcttttgatttataagggattttgccgatttcggcctattggttaaaaaatgagctgatttaacaaaaatttaacgcgaattttaacaaaatattaacgtttacaatttcccaggtggcacttttcggggaaatgtgcgcggaacccctatttgtttatttttctaaatacattcaaatatgtatccgctcatgagacaataaccctgataaatgcttcaataatattgaaaaaggaagagtatgagtattcaacatttccgtgtcgcccttattcccttttttgcggcattttgccttcctgtttttgctcacccagaaacgctggtgaaagtaaaagatgctgaagatcagttgggtgcacgagtgggttacatcgaactggatctcaacagcggtaagatccttgagagttttcgccccgaagaacgttttccaatgatgagcacttttaaagttctgctatgtggcgcggtattatcccgtattgacgccgggcaagagcaactcggtcgccgcatacactattctcagaatgacttggttgagtactcaccagtcacagaaaagcatcttacggatggcatgacagtaagagaattatgcagtgctgccataaccatgagtgataacactgcggccaacttacttctgacaacgatcggaggaccgaaggagctaaccgcttttttgcacaacatgggggatcatgtaactcgccttgatcgttgggaaccggagctgaatgaagccataccaaacgacgagcgtgacaccacgatgcctgtagcaatggcaacaacgttgcgcaaactattaactggcgaactacttactctagcttcccggcaacaattaatagactggatggaggcggataaagttgcaggaccacttctgcgctcggcccttccggctggctggtttattgctgataaatctggagccggtgagcgtgggtctcgcggtatcattgcagcactggggccagatggtaagccctcccgtatcgtagttatctacacgacggggagtcaggcaactatggatgaacgaaatagacagatcgctgagataggtgcctcactgattaagcattggtaactgtcagaccaagtttactcatatatactttagattgatttaaaacttcatttttaatttaaaaggatctaggtgaagatcctttttgataatctcatgaccaaaatcccttaacgtgagttttcgttccactgagcgtcagaccccgtagaaaagatcaaaggatcttcttgagatcctttttttctgcgcgtaatctgctgcttgcaaacaaaaaaaccaccgctaccagcggtggtttgtttgccggatcaagagctaccaactctttttccgaaggtaactggcttcagcagagcgcagataccaaatactgtccttctagtgtagccgtagttaggccaccacttcaagaactctgtagcaccgcctacatacctcgctctgctaatcctgttaccagtggctgctgccagtggcgataagtcgtgtcttaccgggttggactcaagacgatagttaccggataaggcgcagcggtcgggctgaacggggggttcgtgcacacagcccagcttggagcgaacgacctacaccgaactgagatacctacagcgtgagctatgagaaagcgccacgcttcccgaagggagaaaggcggacaggtatccggtaagcggcagggtcggaacaggagagcgcacgagggagcttccagggggaaacgcctggtatctttatagtcctgtcgggtttcgccacctctgacttgagcgtcgatttttgtgatgctcgtcaggggggcggagcctatggaaaaacgccagcaacgcggcctttttacggttcctggccttttgctggccttttgctcacatgttctttcctgcgttatcccctgattctgtggataaccgtattaccgcctttgagtgagctgataccgctcgccgcagccgaacgaccgagcgcagcgagtcagtgagcgaggaagcggaagagcgcccaatacgcaaaccgcctctccccgcgcgttggccgattcattaatgcagctggcacgacaggtttcccgactggaaagcgggcagtgagcgcaacgcaattaatgtgagttagctcactcattaggcaccccaggctttacactttatgcttccggctcgtatgttgtgtggaattgtgagcggataacaatttcacacaggaaacagctatgaccatgattacgccaagcgcgcaattaaccctcactaaagggaacaaaagctggagctgcaagctt

SEQ ID NO: 190 - protein, 220 aa, Artificial Sequence
  Synthetic peptide
  misc_feature (143)..(143): Xaa can be any naturally occurring amino acid
MASAGMQILGVVLTLLGWVNGLVSCALPMWKVTAFIGNSIVVAQVVWEGLWMSCVVQSTGQMQCKVYDSLLALPQDLQAARALCVIALLVALFGLLVYLAGAKCTTCVEEKDSKARLVLTSGIVFVISGVLTLIPVCWTAHAXIRDFYNPLVAEAQKRELGASLYLGWAASGLLLLGGGLLCCTCPSGGSQGPSHYMARYSTSAPAISRGPSEYPTKNYV

SEQ ID NO: 191 - DNA, 68 bp, Artificial Sequence
  Synthetic polynucleotide
cagaaactcatctcagaagaggatctggcagcaaatgatatcctggattacaaggatgacgacgataa

SEQ ID NO: 192 - DNA, 683 bp, Homo sapiens
  ref <308>: NCBI / NM_021195.4
  ref <309>: 2017-06-04
  ref <313>: (1)..(683)
ccgcgatcgccatggcctctgccggaatgcagatcctgggagtcgtcctgacactgctgggctgggtgaatggcctggtctcctgtgccctgcccatgtggaaggtgaccgctttcatcggcaacagcatcgtggtggcccaggtggtgtgggagggcctgtggatgtcctgcgtggtgcagagcaccggccagatgcagtgcaaggtgtacgactcactgctggcgctgccacaggacctgcaggctgcacgtgccctctgtgtcatcgccctccttgtggccctgttcggcttgctggtctaccttgctggggccaagtgtaccacctgtgtggaggagaaggattccaaggcccgcctggtgctcacctctgggattgtctttgtcatctcaggggtcctgacgctaatccccgtgtgctggacggcgcatgccgtcatccgggacttctataaccccctggtggctgaggcccaaaagcgggagctgggggcctccctctacttgggctgggcggcctcaggccttttgttgctgggtggggggttgctgtgctgcacttgcccctcgggggggtcccagggccccagccattacatggcccgctactcaacatctgcccctgccatctctcgggggccctctgagtaccctaccaagaattacgtcacgcgtacgcgg

SEQ ID NO: 193 - DNA, 677 bp, Mus musculas
  ref <308>: NCBI / NM_018777.4
  ref <309>: 2017-08-07
  ref <313>: (1)..(677)
gccgcgatcgccatggcctctactggtctgcaaatcttggggatcgtcctgaccctgcttggctgggtcaacgccctggtgtcctgtgccctgcccatgtggaaggtgaccgccttcatcggcaacagcatcgtcgtggcccagatggtgtgggaggggctgtggatgtcctgtgtggttcagagcactggccagatgcagtgcaaggtgtatgactcactgttggcgctgccccaggacctgcaggctgccagagccctctgtgttgtcaccctcctcattgtcctgcttggcctgctcgtgtacctggctggagccaagtgcactacctgtgtggaagataggaactccaagtctcgtctggtgctcatctctggcatcatctttgtcatttctggggtcctgacgctcattcctgtctgctggactgcccactctatcatccaggacttctacaaccccttggtggctgatgctcaaaagcgggagctgggggcctccctctacctgggctgggcagcctcaggccttttgctgctgggtggagggctactatgctgcgcctgctcttctggagggacccagggacccagacattacatggcctgctattctacatctgtcccacattctcggggaccctccgaatatcccaccaagaattatgtgacgcgtac

SEQ ID NO: 194 - DNA, 683 bp, Artificial Sequence
  Synthetic polynucleotide
cgcgatcgccatggcctctgccggaatgcagatcctgggagtcgtcctgacactgctgggctgggtgaatggcctggtctcctgtgccctgcccatgtggaaggtgaccgctttcatcggcaacagcatcgtggtggcccaggtggtgtgggagggcctgtggatgtcctgcgtggtgcagagcaccggccagatgcagtgcaaggtgtacgactcactgctggcgctgccacaggacctgcaggctgcacgtgccctctgtgtcatcgccctccttgtggccctgttcggcttgctggtctaccttgctggggccaagtgtaccacctgtgtggaggagaaggattccaaggcccgcctggtgctcacctctgggattgtctttgtcatctcaggggtcctgacgctaatccccgtgtgctggacggcgcatgccatcatccgggacttctataaccccctggtggctgaggcccaaaagcgggagctgggggcctccctctacttgggctgggcggcctcaggccttttgttgctgggtggggggttgctgtgctgcacttgcccctcgggggggtcccagggccccagccattacatggcccgctactcaacatctgcccctgccatctctcgggggccctctgagtaccctaccaagaattacgtcacgcgtacgcggc

SEQ ID NO: 195 - DNA, 672 bp, Homo sapiens
  ref <308>: NCBI / NM_020982.3
  ref <309>: 2017-04-15
  ref <313>: (1)..(672)
gccgcgatcgccatggcttcgaccggcttagaactgctgggcatgaccctggctgtgctgggctggctggggaccctggtgtcctgcgccctgcccctgtggaaggtgaccgccttcatcggcaacagcatcgtggtggcccaggtggtgtgggagggcctgtggatgtcctgcgtggtgcagagcacgggccagatgcagtgcaaggtgtacgactcactgctggctctgccgcaggacctgcaggccgcacgtgccctctgtgtcattgccctcctgctggccctgcttggcctcctggtggccatcacaggtgcccagtgtaccacgtgtgtggaggacgaaggtgccaaggcccgtatcgtgctcaccgcgggggtcatcctcctcctcgccggcatcctggtgctcatccctgtgtgctggacggcgcacgccatcatccaggacttctacaaccccctggtggctgaggccctcaagcgggagctgggggcctccctctacctgggctgggcggcggctgcactgcttatgctgggcggggggctcctctgctgcacgtgccccccgccccaggtcgagcggccccgcggacctcggctgggctactccatcccctcccgctcgggtgcatctggactggacaagagggactacgtgacgcgtacg

SEQ ID NO: 196 - DNA, 651 bp, Homo sapiens
  ref <308>: NCBI / NM_001305.4
  ref <309>: 2017-07-10
  ref <313>: (1)..(651)
ccgcgatcgccatggcctccatggggctacaggtaatgggcatcgcgctggccgtcctgggctggctggccgtcatgctgtgctgcgcgctgcccatgtggcgcgtgacggccttcatcggcagcaacattgtcacctcgcagaccatctgggagggcctatggatgaactgcgtggtgcagagcaccggccagatgcagtgcaaggtgtacgactcgctgctggcactgccgcaggacctgcaggcggcccgcgccctcgtcatcatcagcatcatcgtggctgctctgggcgtgctgctgtccgtggtggggggcaagtgtaccaactgcctggaggatgaaagcgccaaggccaagaccatgatcgtggcgggcgtggtgttcctgttggccggccttatggtgatagtgccggtgtcctggacggcccacaacatcatccaagacttctacaatccgctggtggcctccgggcagaagcgggagatgggtgcctcgctctacgtcggctgggccgcctccggcctgctgctccttggcggggggctgctttgctgcaactgtccaccccgcacagacaagccttactccgccaagtattctgctgcccgctctgctgctgccagcaactacgtgacgcgtacgcggc

SEQ ID NO: 197 - DNA, 680 bp, Homo sapiens
  ref <308>: NCBI / NM_001306.3
  ref <309>: 2017-07-10
  ref <313>: (1)..(680)
gccgcgatcgccatgtccatgggcctggagatcacgggcaccgcgctggccgtgctgggctggctgggcaccatcgtgtgctgcgcgttgcccatgtggcgcgtgtcggccttcatcggcagcaacatcatcacgtcgcagaacatctgggagggcctgtggatgaactgcgtggtgcagagcaccggccagatgcagtgcaaggtgtacgactcgctgctggcactgccacaggaccttcaggcggcccgcgccctcatcgtggtggccatcctgctggccgccttcgggctgctagtggcgctggtgggcgcccagtgcaccaactgcgtgcaggacgacacggccaaggccaagatcaccatcgtggcaggcgtgctgttccttctcgccgccctgctcaccctcgtgccggtgtcctggtcggccaacaccattatccgggacttctacaaccccgtggtgcccgaggcgcagaagcgcgagatgggcgcgggcctgtacgtgggctgggcggccgcggcgctgcagctgctggggggcgcgctgctctgctgctcgtgtcccccacgcgagaagaagtacacggccaccaaggtcgtctactccgcgccgcgctccaccggcccgggagccagcctgggcacaggctacgaccgcaaggactacgtcacgcgtac

SEQ ID NO: 198 - protein, 214 aa, Artificial Sequence
  Synthetic peptide
DIVLTQSPATLSVTPGNSVSLSCRASQSIGGNLHWYQQKSHESPRLLIKYASQSISGIPSRFSGSGSGTDFTLSINSVETEDFGMYFCQQSNSWPYTFGGGTKLEIKRADAAPTVSIFPPSSEQLTSGGASVVCFLNNFYPKDINVKWKIDGSERQNGVLNSWTDQDSKDSTYSMSSTLTLTKDEYERHNSYTCEATHKTSTSPIVKSFNRNEC

SEQ ID NO: 199 - protein, 444 aa, Artificial Sequence
  Synthetic peptide
DVQLQESGPSLVKPSQTLSLTCSVTGDSITSDYWSWIRKFPGNRLEYMGYVSYSGSTYYNPSLKSRISITRDTSKNQYYLDLNSVTTEDTATYYCANWDGDYWGQGTLVTVSSAAKTTAPSVYPLAPVCGDTTGSSVTLGCLVKGYFPEPVTLTWNSGSLSSGVHTFPAVLQSDLYTLSSSVTVTSSTWPSQSITCNVAHPASSTKVDKKIEPRGPTIKPCPPCKCPAPNLLGGPSVFIFPPKIKDVLMISLSPIVTCVVVDVSEDDPDVQISWFVNNVEVHTAQTQTHREDYNSTLRVVSALPIQHQDWMSGKEFKCKVNNKDLPAPIERTISKPKGSVRAPQVYVLPPPEEEMTKKQVTLTCMVTDFMPEDIYVEWTNNGKTELNYKNTEPVLDSDGSYFMYSKLRVEKKNWVERNSYSCSVVHEGLHNHHTTKSFSRTPGK

SEQ ID NO: 200 - protein, 220 aa, Artificial Sequence; identical to SEQ ID NO: 190
  Synthetic peptide
  misc_feature (143)..(143): Xaa can be any naturally occurring amino acid

SEQ ID NO: 201 - protein, 220 aa, Artificial Sequence; identical to SEQ ID NO: 190
  Synthetic peptide
  misc_feature (143)..(143): Xaa can be any naturally occurring amino acid

SEQ ID NO: 202-207 - skipped (6 entries)

SEQ ID NO: 208 - DNA, 21 bp, Artificial Sequence
  Synthetic polynucleotide
tccagtgtaagttccacttac

SEQ ID NO: 209 - DNA, 9 bp, Artificial Sequence
  Synthetic polynucleotide
agcacatcc

SEQ ID NO: 210 - DNA, 27 bp, Artificial Sequence
  Synthetic polynucleotide
caccagtatcatcgttccccgctcacg

SEQ ID NO: 211 - DNA, 24 bp, Artificial Sequence
  Synthetic polynucleotide
ggctacacctttactacctacacg

SEQ ID NO: 212 - DNA, 24 bp, Artificial Sequence
  Synthetic polynucleotide
attaatcctagcagtggatatact

SEQ ID NO: 213 - DNA, 27 bp, Artificial Sequence
  Synthetic polynucleotide
gcaaacggggattactacgtcgcttac

SEQ ID NO: 214 - DNA, 18 bp, Artificial Sequence
  Synthetic polynucleotide
gagaatatttacagttat

SEQ ID NO: 215 - DNA, 9 bp, Artificial Sequence
  Synthetic polynucleotide
aatgcaaaa

SEQ ID NO: 216 - DNA, 27 bp, Artificial Sequence
  Synthetic polynucleotide
caacatcattatactgttccgtggacg

SEQ ID NO: 217 - DNA, 24 bp, Artificial Sequence
  Synthetic polynucleotide
ggtttcactttcagtgattactgg

SEQ ID NO: 218 - DNA, 30 bp, Artificial Sequence
  Synthetic polynucleotide
attagattgaaatctgataattatgcaaca

SEQ ID NO: 219 - DNA, 24 bp, Artificial Sequence
  Synthetic polynucleotide
aatgatggccccccctcggggtgt

SEQ ID NO: 220 - DNA, 18 bp, Artificial Sequence
  Synthetic polynucleotide
gagaatatttacagttat

SEQ ID NO: 221 - DNA, 9 bp, Artificial Sequence
  Synthetic polynucleotide
aatgcaaaa

SEQ ID NO: 222 - DNA, 27 bp, Artificial Sequence
  Synthetic polynucleotide
caacatcattatactgttccgtggacg

SEQ ID NO: 223 - DNA, 24 bp, Artificial Sequence
  Synthetic polynucleotide
ggattcactttcagtaattactgg

SEQ ID NO: 224 - DNA, 30 bp, Artificial Sequence; identical to SEQ ID NO: 218
  Synthetic polynucleotide

SEQ ID NO: 225 - DNA, 24 bp, Artificial Sequence
  Synthetic polynucleotide
aatgatggccccccctcggggtgt

SEQ ID NO: 226 - DNA, 33 bp, Artificial Sequence
  Synthetic polynucleotide
cagagccttgtacacagtgatggaaacacctat

SEQ ID NO: 227 - DNA, 9 bp, Artificial Sequence
  Synthetic polynucleotide
aaagtttcc

SEQ ID NO: 228 - DNA, 27 bp, Artificial Sequence
  Synthetic polynucleotide
tctcaaagtacacatgttccttacacg

SEQ ID NO: 229 - DNA, 24 bp, Artificial Sequence
  Synthetic polynucleotide
ggctacacctttactagctacacg

SEQ ID NO: 230 - DNA, 24 bp, Artificial Sequence
  Synthetic polynucleotide
attaatcctagcagtacttatact

SEQ ID NO: 231 - DNA, 30 bp, Artificial Sequence
  Synthetic polynucleotide
tcaagaggggaactgggagggtttgcttac

SEQ ID NO: 232 - DNA, 33 bp, Artificial Sequence
  Synthetic polynucleotide
cagagcattgtacatagtaatggaaacacctat

SEQ ID NO: 233 - DNA, 9 bp, Artificial Sequence
  Synthetic polynucleotide
aaagtttcc

SEQ ID NO: 234 - DNA, 27 bp, Artificial Sequence
  Synthetic polynucleotide
tttcaaggttcacatgttccattcacg

SEQ ID NO: 235 - DNA, 24 bp, Artificial Sequence
  Synthetic polynucleotide
ggatacatattcactcactatatt

SEQ ID NO: 236 - DNA, 24 bp, Artificial Sequence
  Synthetic polynucleotide
attaatccttacaatgatggtact

SEQ ID NO: 237 - DNA, 39 bp, Artificial Sequence
  Synthetic polynucleotide
gcaagatactacggctacccttactattctatggactac

SEQ ID NO: 238 - DNA, 36 bp, Artificial Sequence
  Synthetic polynucleotide
cagagtctgctcaacagtagaacccgaaagaactac

SEQ ID NO: 239 - DNA, 9 bp, Artificial Sequence
  Synthetic polynucleotide
tgggcatcc

SEQ ID NO: 240 - DNA, 24 bp, Artificial Sequence
  Synthetic polynucleotide
aagcaatcttattatctgtacacg

SEQ ID NO: 241 - DNA, 27 bp, Artificial Sequence
  Synthetic polynucleotide
ggctactccatcaccagtggttattac

SEQ ID NO: 242 - DNA, 21 bp, Artificial Sequence
  Synthetic polynucleotide
atcagctacgatggtggcatt

SEQ ID NO: 243 - DNA, 30 bp, Artificial Sequence
  Synthetic polynucleotide
gcaagatttggtaagggggctatggactac

SEQ ID NO: 244 - DNA, 21 bp, Artificial Sequence
  Synthetic polynucleotide
tcaagtgtaagttccagttac

SEQ ID NO: 245 - DNA, 9 bp, Artificial Sequence
  Synthetic polynucleotide
agcacatcc

SEQ ID NO: 246 - DNA, 27 bp, Artificial Sequence
  Synthetic polynucleotide
caccagtatcatcgttccccacccacg

SEQ ID NO: 247 - DNA, 24 bp, Artificial Sequence
  Synthetic polynucleotide
ggttactcattcactggctacacc

SEQ ID NO: 248 - DNA, 24 bp, Artificial Sequence
  Synthetic polynucleotide
attaatccttacaatggtggtact

SEQ ID NO: 249 - DNA, 36 bp, Artificial Sequence
  Synthetic polynucleotide
gcaagaggggtctatgattacgacggatttacttac

SEQ ID NO: 250 - DNA, 33 bp, Artificial Sequence; identical to SEQ ID NO: 226
  Synthetic polynucleotide

SEQ ID NO: 251 - DNA, 9 bp, Artificial Sequence
  Synthetic polynucleotide
aaagtttcc

SEQ ID NO: 252 - DNA, 27 bp, Artificial Sequence
  Synthetic polynucleotide
tctcaaagtacacatgttccttacacg

SEQ ID NO: 253 - DNA, 24 bp, Artificial Sequence
  Synthetic polynucleotide
ggctacacctttactacctacacg

SEQ ID NO: 254 - DNA, 24 bp, Artificial Sequence
  Synthetic polynucleotide
attaatcctcgcagtggttatagt

SEQ ID NO: 255 - DNA, 30 bp, Artificial Sequence; identical to SEQ ID NO: 231
  Synthetic polynucleotide

SEQ ID NO: 256 - DNA, 18 bp, Artificial Sequence
  Synthetic polynucleotide
cagaccattggtacatgg

SEQ ID NO: 257 - DNA, 9 bp, Artificial Sequence
  Synthetic polynucleotide
gctgcagcc

SEQ ID NO: 258 - DNA, 27 bp, Artificial Sequence
  Synthetic polynucleotide
caacaactttacagtattcctcggacg

SEQ ID NO: 259 - DNA, 24 bp, Artificial Sequence
  Synthetic polynucleotide
ggatacagattcactgactacaac

SEQ ID NO: 260 - DNA, 24 bp, Artificial Sequence
  Synthetic polynucleotide
attaaccctaacaatggtggtact

SEQ ID NO: 261 - DNA, 30 bp, Artificial Sequence
  Synthetic polynucleotide
gcaagagattacttgtacttctttgactgc

SEQ ID NO: 262 - DNA, 33 bp, Artificial Sequence
  Synthetic polynucleotide
cagagccttgtacacagtaatggaaacacctat

SEQ ID NO: 263 - DNA, 9 bp, Artificial Sequence
  Synthetic polynucleotide
aaagtttcc

SEQ ID NO: 264 - DNA, 27 bp, Artificial Sequence
  Synthetic polynucleotide
tctcaaattacacatgttccgtacacg

SEQ ID NO: 265 - DNA, 24 bp, Artificial Sequence
  Synthetic polynucleotide
ggttataccttcacagactattca

SEQ ID NO: 266 - DNA, 24 bp, Artificial Sequence
  Synthetic polynucleotide
ataagcactgagactggtgagcca

SEQ ID NO: 267 - DNA, 30 bp, Artificial Sequence
  Synthetic polynucleotide
actagaggtctatggtcctcgtttgcttac

SEQ ID NO: 268 - DNA, 30 bp, Artificial Sequence
  Synthetic polynucleotide
aaaagtgtcagtacatctggctatagttat

SEQ ID NO: 269 - DNA, 9 bp, Artificial Sequence
  Synthetic polynucleotide
cttgcatcc

SEQ ID NO: 270 - DNA, 27 bp, Artificial Sequence
  Synthetic polynucleotide
cagcacagtagggagcttccgctcacg

SEQ ID NO: 271 - DNA, 24 bp, Artificial Sequence
  Synthetic polynucleotide
ggattcactttcagtagctttgga

SEQ ID NO: 272 - DNA, 24 bp, Artificial Sequence
  Synthetic polynucleotide
attagtagtgacagtaggaccatc

SEQ ID NO: 273 - DNA, 33 bp, Artificial Sequence
  Synthetic polynucleotide
gcaagagactacggtagaacctacgaggcttac

SEQ ID NO: 274 - DNA, 18 bp, Artificial Sequence
  Synthetic polynucleotide
caggacattggaggaaat

SEQ ID NO: 275 - DNA, 9 bp, Artificial Sequence
  Synthetic polynucleotide
tccacatcc

SEQ ID NO: 276 - DNA, 27 bp, Artificial Sequence
  Synthetic polynucleotide
ctacagcgtaatgcgtatccgctcact

SEQ ID NO: 277 - DNA, 24 bp, Artificial Sequence
  Synthetic polynucleotide
ggattcactttcagtagttatgcc

SEQ ID NO: 278 - DNA, 21 bp, Artificial Sequence
  Synthetic polynucleotide
attagaagtggtggtaccacc

SEQ ID NO: 279 - DNA, 36 bp, Artificial Sequence
  Synthetic polynucleotide
gcaaaagtgggcggtaacccctatcctatggactac

SEQ ID NO: 280 - DNA, 21 bp, Artificial Sequence
  Synthetic polynucleotide
tcaagtataagttccaattac

SEQ ID NO: 281 - DNA, 9 bp, Artificial Sequence
  Synthetic polynucleotide
aggacatcc

SEQ ID NO: 282 - DNA, 27 bp, Artificial Sequence
  Synthetic polynucleotide
cagcagggtagtagtataccgctcacg

SEQ ID NO: 283 - DNA, 24 bp, Artificial Sequence
  Synthetic polynucleotide
ggatacgccttcagtaattacttg

SEQ ID NO: 284 - DNA, 24 bp, Artificial Sequence
  Synthetic polynucleotide
attaatcctggaagtggtggtact

SEQ ID NO: 285 - DNA, 45 bp, Artificial Sequence
  Synthetic polynucleotide
gcaagatcatacttcggtagaagctacccctatactatggactac

SEQ ID NO: 286 - DNA, 30 bp, Artificial Sequence
  Synthetic polynucleotide
caaagtgttgattatgatggtgataattat

SEQ ID NO: 287 - DNA, 9 bp, Artificial Sequence
  Synthetic polynucleotide
gctgcatcc

SEQ ID NO: 288 - DNA, 27 bp, Artificial Sequence
  Synthetic polynucleotide
cagcaaagtaatgaggatccattcacg

SEQ ID NO: 289 - DNA, 24 bp, Artificial Sequence
  Synthetic polynucleotide
ggctacacattcactgattatgct

SEQ ID NO: 290 - DNA, 24 bp, Artificial Sequence
  Synthetic polynucleotide
attagtacatactctggtaataca

SEQ ID NO: 291 - DNA, 39 bp, Artificial Sequence
  Synthetic polynucleotide
gcaagaaggggcgattacagcctctatgctatggactac

SEQ ID NO: 292 - DNA, 36 bp, Artificial Sequence
  Synthetic polynucleotide
caaagtgttttattcagttcaaatcagaaaaactac

SEQ ID NO: 293 - DNA, 9 bp, Artificial Sequence
  Synthetic polynucleotide
tgggcatcc

SEQ ID NO: 294 - DNA, 24 bp, Artificial Sequence
  Synthetic polynucleotide
catcaatacctctcctcgcgcacg

SEQ ID NO: 295 - DNA, 24 bp, Artificial Sequence
  Synthetic polynucleotide
ggattcactttcagtagctttgga

SEQ ID NO: 296 - DNA, 24 bp, Artificial Sequence
  Synthetic polynucleotide
attagtagtgacagtaggaccatc

SEQ ID NO: 297 - DNA, 33 bp, Artificial Sequence; identical to SEQ ID NO: 273
  Synthetic polynucleotide

SEQ ID NO: 298 - DNA, 30 bp, Artificial Sequence
  Synthetic polynucleotide
gaaagtgttgataattatggcattagtttt

SEQ ID NO: 299 - DNA, 9 bp, Artificial Sequence
  Synthetic polynucleotide
gctgcatcc

SEQ ID NO: 300 - DNA, 27 bp, Artificial Sequence
  Synthetic polynucleotide
cagcaaagtaaggaggttccgctcacg

SEQ ID NO: 301 - DNA, 24 bp, Artificial Sequence
  Synthetic polynucleotide
ggattccctttcagtagctctgcc

SEQ ID NO: 302 - DNA, 21 bp, Artificial Sequence
  Synthetic polynucleotide
attaatagtgatggtaacacc

SEQ ID NO: 303 - DNA, 39 bp, Artificial Sequence
  Synthetic polynucleotide
acaagaaacggggactataggtacgacgagtttgcttac

SEQ ID NO: 304 - DNA, 21 bp, Artificial Sequence
  Synthetic polynucleotide
tcaagtgtaagttccagttac

SEQ ID NO: 305 - DNA, 9 bp, Artificial Sequence
  Synthetic polynucleotide
agcacatcc

SEQ ID NO: 306 - DNA, 27 bp, Artificial Sequence
  Synthetic polynucleotide
caccagtatcatcgttccccacccacg

SEQ ID NO: 307 - DNA, 24 bp, Artificial Sequence
  Synthetic polynucleotide
ggctacacctttactggctactgg

SEQ ID NO: 308 - DNA, 24 bp, Artificial Sequence
  Synthetic polynucleotide
attaatcctagcactggttatact

SEQ ID NO: 309 - DNA, 36 bp, Artificial Sequence
  Synthetic polynucleotide
gcaagagaggggattactactgtgctggttgactac

SEQ ID NO: 310 - DNA, 36 bp, Artificial Sequence; identical to SEQ ID NO: 292
  Synthetic polynucleotide

SEQ ID NO: 311 - DNA, 9 bp, Artificial Sequence
  Synthetic polynucleotide
tgggcatcc

SEQ ID NO: 312 - DNA, 24 bp, Artificial Sequence
  Synthetic polynucleotide
catcaatacctctcctcgcgcacg

SEQ ID NO: 313 - DNA, 24 bp, Artificial Sequence
  Synthetic polynucleotide
ggttactctttcactggctacaat

SEQ ID NO: 314 - DNA, 24 bp, Artificial Sequence
  Synthetic polynucleotide
attgatccttactatggtggttct

SEQ ID NO: 315 - DNA, 42 bp, Artificial Sequence
  Synthetic polynucleotide
gcaagagagaggtcgggctacgttttctctgctatggactac

SEQ ID NO: 316 - DNA, 36 bp, Artificial Sequence; identical to SEQ ID NO: 292
  Synthetic polynucleotide

SEQ ID NO: 317 - DNA, 9 bp, Artificial Sequence
  Synthetic polynucleotide
tgggcatcc

SEQ ID NO: 318 - DNA, 24 bp, Artificial Sequence
  Synthetic polynucleotide
catcaatacctctcctcgcgcacg

SEQ ID NO: 319 - DNA, 24 bp, Artificial Sequence
  Synthetic polynucleotide
ggttactcattcactggctacacc

SEQ ID NO: 320 - DNA, 24 bp, Artificial Sequence
  Synthetic polynucleotide
attaatccttacaatggtgttact

SEQ ID NO: 321 - DNA, 48 bp, Artificial Sequence
  Synthetic polynucleotide
acaagagatcccctttactacggctacagggactctactatggactac

SEQ ID NO: 322 - DNA, 33 bp, Artificial Sequence; identical to SEQ ID NO: 226
  Synthetic polynucleotide

SEQ ID NO: 323 - DNA, 9 bp, Artificial Sequence
  Synthetic polynucleotide
aaagtttcc

SEQ ID NO: 324 - DNA, 27 bp, Artificial Sequence
  Synthetic polynucleotide
tctcaaagtacacatgttccttacacg

SEQ ID NO: 325 - DNA, 24 bp, Artificial Sequence
  Synthetic polynucleotide
ggctacacctttactagctacacg

SEQ ID NO: 326 - DNA, 24 bp, Artificial Sequence
  Synthetic polynucleotide
attaatcctagcagtacgtatact

SEQ ID NO: 327 - DNA, 30 bp, Artificial Sequence; identical to SEQ ID NO: 231
  Synthetic polynucleotide

SEQ ID NO: 328 - DNA, 18 bp, Artificial Sequence
  Synthetic polynucleotide
cagggcattagaggtaat

SEQ ID NO: 329 - DNA, 9 bp, Artificial Sequence
  Synthetic polynucleotide
tccacatcc

SEQ ID NO: 330 - DNA, 27 bp, Artificial Sequence
  Synthetic polynucleotide
ctacagcgtaatgcgtatcctctcacg

SEQ ID NO: 331 - DNA, 24 bp, Artificial Sequence
  Synthetic polynucleotide
ggattcactttcagtagttttgcc

SEQ ID NO: 332 - DNA, 21 bp, Artificial Sequence
  Synthetic polynucleotide
attagaagtggtggtattacc

SEQ ID NO: 333 - DNA, 39 bp, Artificial Sequence
  Synthetic polynucleotide
gcaagagttagtacggctacgtactatggtatggactac

SEQ ID NO: 334 - DNA, 325 bp, Artificial Sequence
  Synthetic polynucleotide
caaattgttctcacccagtctccagcaatcatgtctgcatctctaggggaacgggtcaccatgacctgcactgccagctccagtgtaagttccacttactttcactggtaccaacagaagccaggatcctcccccaaactctggatttatagcacatccaacctggcttctggagtcccacgtcgcttcagtggcagtgcgtctgggacctcttactctctcacaatcagcagcatggaggctgaagatgctgccacttattattgccaccagtatcatcgttccccgctcacgttcggtgctgggaccaagctggagctgaaac

SEQ ID NO: 335 - DNA, 349 bp, Artificial Sequence
  Synthetic polynucleotide
caggtccagctgcagcagtctgcagctgaactggcaagacctggggcctcagtgaagatgtcctgcaaggcttctggctacacctttactacctacacgatgcactgggtaaaacagaggcctggacagggtctggaatggattggattcattaatcctagcagtggatatactgactacaatcagaagttcaaggacaggaccacattgactgcagacaaatcctccagcacagtctacatgcaactgagtagcctgacatctgaggactctgcggtctattactgtgcaaacggggattactacgtcgcttactggggccaagggactctggtcactgtctctgcag

SEQ ID NO: 336 - DNA, 322 bp, Artificial Sequence
  Synthetic polynucleotide
gacatccagatgactcagtctccagcctccctatctgcatctgtgggagaaactgtcaccatcacatgtcgaataagcgagaatatttacagttatttagcatggtatcagcagaaacagggaaaatctcctcagctcctggtctataatgcaaaaatcttagtagaaggtgtgccatcaaggttcagtggcagtggatcaggcacacagttttctctgaagatcaacagcctgcagcctgaagattttgggaattattactgtcaacatcattatactgttccgtggacgttcggtggaggcaccaaactggaaatcaaac

SEQ ID NO: 337 - DNA, 352 bp, Artificial Sequence
  Synthetic polynucleotide
gaagtgaagcttgaggagtctggaggaggcttggtgcaacctggaggatccatgaaactctcctgtgttgcctctggtttcactttcagtgattactggatgaactgggtccgccagtctccagagaaggggcttgaatgggttgctcaaattagattgaaatctgataattatgcaacacattatgcggagtctgtgaaagggaggttcaccatctcaagagatgattccaaaagaagtgtctacctgcaaatgaacaacttaagggctgaagacactggaacttattactgcaatgatggccccccctcggggtgttggggccaaggcaccactctcatagtctcctcag

SEQ ID NO: 338 - DNA, 322 bp, Artificial Sequence
  Synthetic polynucleotide
gacatccagatgactcagtctccagcctccctatctgcatctgtgggagaaactgtcaccatcacatgtcgaataagtgagaatatttacagttatttagcatggtatcagcagaaacagggaaaatctcctcagctcctggtctataatgcaaaaatcttagtagaaggtgtgccatcaaggttcagtggcagtggatcaggcacacagttttctctgaagatcaacagcctgcagcctgaagattttgggaattattactgtcaacatcattatactgttccgtggacgttcggtggaggcaccaaactggaaatcaaac

SEQ ID NO: 339 - DNA, 352 bp, Artificial Sequence
  Synthetic polynucleotide
gaagtgaagcttgaggagtctggaggaggcttggtgcaacctggaggatccatgaaactctcctgtgttgcctctggattcactttcagtaattactggatgaactgggtccgccagtctccagagaaggggcttgaatgggttgctcaaattagattgaaatctgataattatgcaacacattatgcggagtctgtgaaagggaggttcaccatctcaagagatgattccaaaagaagtgtctacctgcaaatgaacaacttaagggctgaagacactggaacttattactgcaatgatggccccccctcggggtgttggggccaaggcaccactctcatagtctcctcag

SEQ ID NO: 340 - DNA, 337 bp, Artificial Sequence
  Synthetic polynucleotide
gatgttgtgatgacccaaactccactctccctgcctgtcagtcttggagatcaagcctccatctcttgcagatctagtcagagccttgtacacagtgatggaaacacctatttaaattggtacctgcagaagccaggccagtctccaaagctcctgatctacaaagtttccaaccgtttttctggggtcccagacaggttcagtggcagtggatcagggacagatttcacactcaagatcaggagagtggaggctgaggatctgggagtttatttctgctctcaaagtacacatgttccttacacgttcggaggggggaccaagctggaaataaaac

SEQ ID NO: 341 - DNA, 352 bp, Artificial Sequence
  Synthetic polynucleotide
caggtccagttgcagcagtctggggctgaactggcaagacctggggcctcagtgaagatgtcctgcaaggcttctggctacacctttactagctacacgatgcactggataaaacagagacctggacagggtcaggaatggattggatacattaatcctagcagtacttatactcattacattaagaaattcaaggacaaggccacattgactgcagacaaatcctccagcacagcctacatgcaactgcgcagcctgacatctgaggactctgcagtctattactgttcaagaggggaactgggagggtttgcttactggggccaagggactctggtcactgtctctgcag

SEQ ID NO: 342 - DNA, 337 bp, Artificial Sequence
  Synthetic polynucleotide
gatgttttgatgacccaaactccactctccctgcctgtcagtcttggagatcaaccctccatctcttgcagatctagtcagagcattgtacatagtaatggaaacacctatttagattggtacctgcagaaaccaggccagtctccaaagctcctgatctacaaagtttccaaccgattttctggggtcccagacaggttcagtggcagtggatcagggacagatttcacactcaagatcagcagagtggaggctgaggatctgggagtttattactgctttcaaggttcacatgttccattcacgttcggctcggggacaaggttggaaataaaac

SEQ ID NO: 343 - DNA, 361 bp, Artificial Sequence
  Synthetic polynucleotide
gaagtccagctgcagcagtctggacctgagctggtaaagcctggggcttcagtgaagatgtcctgcaaggcttctggatacatattcactcactatattatgcactgggtgaagcagaagcctgggcagggccttgagtggattggatgtattaatccttacaatgatggtactaagtacaatgagaagttcaaaggcaaggccacactgacttcagacaaatcctccagcacagcctacatggagctcagcagcctgacctctgaggactctgcggtctattactgtgcaagatactacggctacccttactattctatggactactggggtcaaggaacctcagtcaccgtctcctcag

SEQ ID NO: 344 - DNA, 337 bp, Artificial Sequence
  Synthetic polynucleotide
gccattgtgatgttccagtctccatcctccctggttgtgtcagcaggagagaaggtcactatgagctgcaaatccagtcagagtctgctcaacagtagaacccgaaagaactacttggcttggtaccagcagaaaccagggcagtctcctaaactgctgatctactgggcatccactagggaatctggggtccctgatcgcttcacaggcagtggatctgggacagatttcactctcaccatcagcagtgtgcaggctgaagacctggcagtttattactgcaagcaatcttattatctgtacacgttcggaggggggaccaagctggaaataaaac

SEQ ID NO: 345 - DNA, 352 bp, Artificial Sequence
  Synthetic polynucleotide
gatgtgcagcttcaggagtcaggacctggcctcgtgaaatcttctcagtctctgtctctcacctgctctgtcactggctactccatcaccagtggttattactggaaatggatccggcagtttccaggaaacaaactggaatggatgggctacatcagctacgatggtggcattaactacaacccatctctcaaaaatcgaatctccatcactcgtgacacatctaagaaccagtttttcctgaagttgaattctgtgactactgaggacacagccaaatattactgtgcaagatttggtaagggggctatggactactggggtcaaggaacctcagtcaccgtctcctcag

SEQ ID NO: 346 - DNA, 325 bp, Artificial Sequence
  Synthetic polynucleotide
caaattgttctcacccagtctccagcaatcatgtctgcatctctgggggaccgggtcaccatgacctgcactgccagctcaagtgtaagttccagttacttgcactggtaccagcagaagccaggatcctcccccaaactctggatttatagcacatccaacctggcttctggagtcccagctcgcttcagtggcagtgggtctgggacctcttactctctcacaatcagcagcatggaggctgaagatgctgccacttattactgccaccagtatcatcgttccccacccacgttcggctcggggacaaagttggaaataaaac

SEQ ID NO: 347 - DNA, 358 bp, Artificial Sequence
  Synthetic polynucleotide
gaggtccagctgcaacagtctggacctgagctggtgaagcctggagcttcaatgaagatatcctgcaaggcttctggttactcattcactggctacaccatgaactgggtgaagcagagccatggaaagaaccttgagtggattggacttattaatccttacaatggtggtactaactacaaccagaagttcaagggcaaggccacattaactgtagacaagtcatccagcacagcctacatggagctcctcagtctgacatctgaggactctgcagtctattactgtgcaagaggggtctatgattacgacggatttacttactggggccaagggactctggtcactgtctctgcag

SEQ ID NO: 348 - DNA, 337 bp, Artificial Sequence
  Synthetic polynucleotide
gatgttgtgatgacccaaactccactctccctgcctgtcagtcttggagatcaagcctccatctcttgcagatctagtcagagccttgtacacagtgatggaaacacctatttatattggtacctgcagaagccaggccagtctccaaagctcctgatctacaaagtttccaaccgattttctggggtcccagacaggttcagtggcagtggatcagggacagatttcacactcaagatcagcagagtggaggctgaggatctgggagtttatttctgctctcaaagtacacatgttccttacacgttcggaggggggaccaagctggaaataaaac

SEQ ID NO: 349 - DNA, 352 bp, Artificial Sequence
  Synthetic polynucleotide
caggtccagctgcagcagtctggggctgaactggcaagacctggggcctcagtgaagatgtcctgcaaggcttctggctacacctttactacctacacgatgcactggttaaaacagaggcctggacagggtctggaatggattggatacattaatcctcgcagtggttatagtaattacaatcagaagttcaaggacaaggccacattgactgcagacaagtcctccaacacagcctacatgcaactgaacaccctgacatctgaggactctaaagtctattactgttcaagaggggaactgggagggtttgcttactggggccaagggactctggtcactgtctctgcag

SEQ ID NO: 350 - DNA, 322 bp, Artificial Sequence
  Synthetic polynucleotide
gacattcagatgacccagtctcctgcctcccagtctgcatctctgggagaaagtgtcaccatcacatgcctggcaagtcagaccattggtacatggttagcatggtatcagcagaaaccagggaaatctcctcagctcctgatttatgctgcagccagcttggcagatggggtcccatcaaggttcagtggtagtggatctggcacaagattttctttcaagatcagcagcctacaggctgaagattttgtaagttattactgtcaacaactttacagtattcctcggacgttcggtggaggcaccaagctggaaatcaaac

SEQ ID NO: 351 - DNA, 352 bp, Artificial Sequence
  Synthetic polynucleotide
gaggtccagctgcaacagtctggacctgagctggtgaagcctggggcttcagtgaagatgtcctgcaaggcttctggatacagattcactgactacaacatgcactgggtgaagcagagccatggaaagagccttgagtggattggatatattaaccctaacaatggtggtactaactacaaccaaaacttcaagggcaaggccacattgactgtgaacaagtcctccagcacagcctacatggagctccgcagcctgacatcggaggattctgcagcctattactgtgcaagagattacttgtacttctttgactgctggggccaaggcaccactctcacagtctcctcag

SEQ ID NO: 352 - DNA, 337 bp, Artificial Sequence
  Synthetic polynucleotide
gatgttgtgatgacccaaactccactctccctgcctgtcagtcttggagatcaagcctccatctcttgcagagctagtcagagccttgtacacagtaatggaaacacctatttacattggttcctgcagaagccaggccagtctccaaagctcctgatctacaaagtttccaaccgattttctggggtcccagacaggttcagtggcagtggatcacggacagatttcacactcaagatcagcagagtggaggctgaggatctgggagtttatttctgctctcaaattacacatgttccgtacacgttcggaggggggaccaagctggaaataaaac

SEQ ID NO: 353 - DNA, 352 bp, Artificial Sequence
  Synthetic polynucleotide
caaatccagttggtgcagtctggacctgcgctgaagaagcctggagagacagtcaagatctcctgcaaggcttctggttataccttcacagactattcaatgcactggataaagcaggctccaggaaagggtttaaagtggatgggctggataagcactgagactggtgagccaacatatgcagatggcttcaagggacggtttgacttctctttggaaacctctgccgacactgcctatttgtccatcaacaacctcacaaatgaggacacggctacatatttctgtactagaggtctatggtcctcgtttgcttactggggccaagggactctggtcactgtctctgcag

SEQ ID NO: 354 - DNA, 334 bp, Artificial Sequence
  Synthetic polynucleotide
gacattgtgctgacacagtctcctgcttccttagctgtatctctggggcagagggccaccatctcatgcagggccagcaaaagtgtcagtacatctggctatagttatatacactggtaccaacagaaaccaggacagccacccaaactcctcatctatcttgcatccaacctagaatctggggtccctgccaggttcagtggcagtgggtctgggacagacttcaccctcaacatccatcctgtggaggaggaggatgctgcaacctattactgtcagcacagtagggagcttccgctcacgttcggtgctgggaccaagctggagctgaaac

SEQ ID NO: 355 - DNA, 355 bp, Artificial Sequence
  Synthetic polynucleotide
gatgtgcagctggtggagtctgggggaggcttggtgcagcctagagggtcccggaaactctcctgtgcagcctctggattcactttcagtagctttggaatgcactgggttcgtcaggctccagagaaggggctggagtgggtcgcatacattagtagtgacagtaggaccatctattatgcagacacagtgaagggccgattcaccatctccagagacaatcccacgaacaccctgttcctgcaaatgaccagtctcaggtctgaggacacggccatgtattactgtgcaagagactacggtagaacctacgaggcttactggggccaagggactctggtcactgtctctgcag

SEQ ID NO: 356 - DNA, 322 bp, Artificial Sequence
  Synthetic polynucleotide
gacatccagatgattcagtctccatcgtccatgtttgcctctctgggagacagagtcagtctctcttgtcgggctagtcaggacattggaggaaatttagactggtatcagcagaaaccaggtggaactattaaactcctgatctactccacatccaatttaaattctggtgtcccatcaaggttcagtggcagtgggtctgggtcagattattctctcaccatcaccagcctggagtctgaagattttgcagactattactgtctacagcgtaatgcgtatccgctcactttcggtgctgggaccaagctggagctgaaac

SEQ ID NO: 357 - DNA, 355 bp, Artificial Sequence
  Synthetic polynucleotide
gaagtgaaactgatggagtctgggggagacttagtgaagcctggagggtccctgaaactctcctgtgcagcctctggattcactttcagtagttatgccatgtcttgggttcgccagactccagagaagaggctggagtgggtcgcgtccattagaagtggtggtaccacctactatccagacagtgtgaagggccgattcaccatctccagagataatgccaggaacatcctgtacctgcgaatgagtagtctgaggtctgaggacacggccatatattactgtgcaaaagtgggcggtaacccctatcctatggactactggggtcaaggaacctcagtcaccgtctcctcag

SEQ ID NO: 358 - DNA, 325 bp, Artificial Sequence
  Synthetic polynucleotide
gaaattgtgctcacccagtctccaaccaccatggctgcatctcccggggagaagatcactatcacctgcagtgccagctcaagtataagttccaattacttgcattggtatcagcagaagccaggattctcccctaaactcttgatttataggacatccaatctggcttctggagtcccagctcgcttcagtggcagtgggtctgggacctcttactctctcacaattggcaccatggaggctgaagatgttgccacttactactgccagcagggtagtagtataccgctcacgttcggtgctgggaccaagctggagctgaaac

SEQ ID NO: 359 - DNA, 367 bp, Artificial Sequence
  Synthetic polynucleotide
caggtccagctgcagcagtctggagctgagctggtaaggcctgggacttcagtgaaggtgtcctgcaaggcttctggatacgccttcagtaattacttgatagagtgggttaagcagaggcctggacagggccttgagtggattggagtgattaatcctggaagtggtggtactaactacaatgagaagttcaagggcaaggcaacaatgactgcagacaaatcctccagcactgcctacatgcacctcagcaacctgacatctgaggactctgtggtctatttctgtgcaagatcatacttcggtagaagctacccctatactatggactactggggtcaaggaacctcagtcaccgtctcctcag

SEQ ID NO: 360 - DNA, 334 bp, Artificial Sequence
  Synthetic polynucleotide
gatattgtgctgacccaatctccagcttctttggctgtgtctctagggcagagggccaccatctcctgcaaggccagccaaagtgttgattatgatggtgataattatgtgaactggtaccaacagaaagtaggacagccacccaaactcctcatctctgctgcatccaatctagaatctgggatcccagccaggtttagtggcagtgggtctgggacagacttcaccctcaacatccatcctgtggaggaggaggatgctgcaacctattactgtcagcaaagtaatgaggatccattcacgttcggctcggggacaaagttggaaataaaac

SEQ ID NO: 361 - DNA, 361 bp, Artificial Sequence
  Synthetic polynucleotide
caggtccagctgcagcagtctgggcctgagctggtgaggcctggggtctcagtgaagatttcctgcaagggttccggctacacattcactgattatgctatgcactgggtgaagcagagtcatgcaaagagtctagagtggattggagttattagtacatactctggtaatacaaactacaaccagaagtttcaggacaaggccaccatgactgtagacaaatcctccagcacagcctatatggcacttgccagattgacatctgacgattctgccatctattactgtgcaagaaggggcgattacagcctctatgctatggactactggggtcaaggaacctcagtcaccgtctcctcag

SEQ ID NO: 362 - DNA, 337 bp, Artificial Sequence
  Synthetic polynucleotide
aacattatgatgacacagtcgccatcatctctggctgtgtctgcaggagaaaaggtcactatgagctgtaagtccagtcaaagtgttttattcagttcaaatcagaaaaactacttggcctggtaccagcagaaaccagggcagtctcctagactgctgatctactgggcatccactagggaatctggtgtccctgatcgcttcacaggcagtggatctgggacagattttactcttaccatcagcaatgttcaagctgaagacctggcagtttattactgtcatcaatacctctcctcgcgcacgttcggtgctgggaccaagctggagctgaaac

SEQ ID NO: 363 - DNA, 355 bp, Artificial Sequence; identical to SEQ ID NO: 355
  Synthetic polynucleotide

SEQ ID NO: 364 - DNA, 334 bp, Artificial Sequence
  Synthetic polynucleotide
gacattgtgctgacccaatctccagcttctttggctctgtctctagggcagagggccaccatctcctgcagagccagcgaaagtgttgataattatggcattagttttatgaactggttccaacagaaacccggacagccacccaaactcctcatctatgctgcatccaaccaaggatccggggtccctgccaggtttagtggcagtgggtctgggacagacttcagcctcaacatccatcctatggaggaggatgatactgcaatgtatttctgtcagcaaagtaaggaggttccgctcacgttcggtgctgggaccaagctggagctgaaac

SEQ ID NO: 365 - DNA, 358 bp, Artificial Sequence
  Synthetic polynucleotide
gaagtgaggctggtggagtctgggggaggcttgatgcagcctggagggtccctgaaactcccctgtgcagcctctggattccctttcagtagctctgccatgtcttgggttcgccagactccagagaagaggctggagtgggtcgcatccattaatagtgatggtaacacctactatcccgacagtgtgaagggccgattcaccatctccagagatagtgccaggaacatcctgtacctccaaatgagcagtctgaggtctgaggacacggccatgtattactgtacaagaaacggggactataggtacgacgagtttgcttactggggccaagggactctggtcactgtctctgcag

SEQ ID NO: 366 - DNA, 325 bp, Artificial Sequence
  Synthetic polynucleotide
caaattgttctcacccagtctccagcaatcatgtctgcatctctaggggaacgggtcaccatgacctgcactgccagctcaagtgtaagttccagttacttgcactggtaccagcagaagccaggatcctcccccaaactctggatttatagcacatccaacctggcttctggagtcccagctcgcttcagtggcagtgggtctgggacctcttactctctcacaatcagcagcatggaggctgaagatgctgccacttattactgccaccagtatcatcgttccccacccacgttcggagctgggaccaagctggagctgaaac

SEQ ID NO: 367 - DNA, 358 bp, Artificial Sequence
  Synthetic polynucleotide
caggtccagcttcagcagtctggggctgaactggcaaaacctggggcctcagtgaagatgtcctgcaaggcttctggctacacctttactggctactggatgcactgggtaaaacagaggcctggacagggtctggaatggcttggatacattaatcctagcactggttatactgagtccaatcagaagttcaaggacaaggccacattgactgcagacaaatcctccaccacagcctacatgcaactgagaagcctgacacctgaggactctgcagtctattactgtgcaagagaggggattactactgtgctggttgactactggggccaaggcaccactctcacagtctcctcag

SEQ ID NO: 368 - DNA, 337 bp, Artificial Sequence; identical to SEQ ID NO: 362
  Synthetic polynucleotide

SEQ ID NO: 369 - DNA, 364 bp, Artificial Sequence
  Synthetic polynucleotide
caggtgcagctgaagcagtctggacctgagctggagaagcctggcgcttcagtgaagatatcctgcaaggcttctggttactctttcactggctacaatatgaactgggtgaagcagagcaatggaaagagccttgagtggattggaaatattgatccttactatggtggttctacctacaaccagaagttcacgggcaaggccacattgactgtagacaaatcctccagcacagcctacatgcagctcaagagcctgacatctgaggactctgcagtgtattactgtgcaagagagaggtcgggctacgttttctctgctatggactactggggtcaaggaacctcagtcaccgtctcctcag

SEQ ID NO: 370 - DNA, 337 bp, Artificial Sequence; identical to SEQ ID NO: 362
  Synthetic polynucleotide

SEQ ID NO: 371 - DNA, 370 bp, Artificial Sequence
  Synthetic polynucleotide
gaggtccagctgcaacagtctggacctgagctggtgaagcctggaggttcaatgaagatatcctgcaaggcttctggttactcattcactggctacaccatgaactgggtgaagcggagccatggaaagaaccttgagtggattggacttattaatccttacaatggtgttactacctacaaccagaacttcaagggcaaggccacattagctgtagacaagtcatccagcacagcctacatggagctcctcggtctgacatctgaggactctgcagtctattactgtacaagagatcccctttactacggctacagggactctactatggactactggggtcaaggaacctcagtcaccgtctcctcag

SEQ ID NO: 372 - DNA, 337 bp, Artificial Sequence; identical to SEQ ID NO: 340
  Synthetic polynucleotide

SEQ ID NO: 373 - DNA, 352 bp, Artificial Sequence
  Synthetic polynucleotide
gaggtccagctgcagcagtctggggctgaactggcaagacctggggcctcagtgaagatgtcctgcaaggcttctggctacacctttactagctacacgatgcactggataaaacagagacctggacagggtcaggaatggattggatacattaatcctagcagtacgtatactcattacattaagaagttcaaggacaaggccacattgactgcagacaaatcctccagcacagcctacatgcaactgcgcagcctgacatctgaggactctgcagtctattactgttcaagaggggaactgggagggtttgcttactggggccaagggactctggtcactgtctctgcag

SEQ ID NO: 374 - DNA, 322 bp, Artificial Sequence
  Synthetic polynucleotide
gacatccagatgattcagtctccatcgtccatgtttgcctctctgggagacagagtcagtctctcttgtcgggctagtcagggcattagaggtaatttagactggtatcagcagaaaccaggtggaactattaaactcctgatctactccacatccattttaaattctggtgtcccatcaaggttcagtggcagtgggtctgggtcagattattctctcaccatcaccagcctagagtctgaagattttgcagactattactgtctacagcgtaatgcgtatcctctcacgttcggttctgggaccaagctggagctgaaac

SEQ ID NO: 375 - DNA, 358 bp, Artificial Sequence
  Synthetic polynucleotide
gaagtgaagttggtggagtctgggggaggcttaatgaagcctggagggtccctgaaactctcctgtgcggcctctggattcactttcagtagttttgccttgtcttgggttcgccagactccagagaagaggctggagtgggtcgcatccattagaagtggtggtattacctaccatgcagacagtgtgaagggccgattcaccatctccagagataatgccgggaacatcctgtacctgcaaatgaacagtctgaggtctgaggacacggccatgtatttctgtgcaagagttagtacggctacgtactatggtatggactactggggtcaaggaacctcagtcaccgtctcctcag

SEQ ID NO: 376 - protein, 116 aa, Artificial Sequence
  Synthetic peptide
QVQLVQSGAEVKKPGASVKVSCKASGYTFTTYTMHWVRQAPGQGLEWMGFINPSSGYTDYAQKFQGRVTMTRDTSTSTVYMELSSLRSEDTAVYYCARGDYYVAYWGQGTLVTVSS

SEQ ID NO: 377 - protein, 116 aa, Artificial Sequence
  Synthetic peptide
QVQLVQSGAEVKKPGASVKVSCKASGYTFTTYTMHWVRQAPGQGLEWMGFINPSSGYTDYAQKFQGRVTMTADTSTSTVYMELSSLRSEDTAVYYCANGDYYVAYWGQGTLVTVSS

SEQ ID NO: 378 - protein, 116 aa, Artificial Sequence
  Synthetic peptide
QVQLVQSGAEVKKPGASVKMSCKASGYTFTTYTMHWVRQAPGQGLEWIGFINPSSGYTDYAQKFQGRVTLTADTSTSTVYMELSSLRSEDTAVYYCANGDYYVAYWGQGTLVTVSS

SEQ ID NO: 379 - protein, 116 aa, Artificial Sequence
  Synthetic peptide
QVQLVQSGAEVKKPGASVKMSCKASGYTFTTYTMHWVRQAPGQGLEWIGFINPSSGYTDYAQKFQGRVTLTADKSTSTVYMELSSLRSEDTAVYYCANGDYYVAYWGQGTLVTVSS

SEQ ID NO: 380 - protein, 108 aa, Artificial Sequence
  Synthetic peptide
DIQMTQSPSSLSASVGDRVTITCTASSSVSSTYFHWYQQKPGKAPKLLIYSTSNLASGVPSRFSGSGSGTDFTLTISSLQPEDFATYYCHQYHRSPLTFGQGTKLEIK

SEQ ID NO: 381 - protein, 108 aa, Artificial Sequence
  Synthetic peptide
DIQMTQSPSSLSASVGDRVTITCTASSSVSSTYFHWYQQKPGKAPKLLIYSTSNLASGVPSRFSGSGSGTDYTLTISSLQPEDFATYYCHQYHRSPLTFGQGTKLEIK

SEQ ID NO: 382 - protein, 108 aa, Artificial Sequence
  Synthetic peptide
DIQLTQSPSSLSASVGDRVTMTCTASSSVSSTYFHWYQQKPGKAPKLLIYSTSNLASGVPSRFSGSGSGTDYTLTISSMQPEDAATYYCHQYHRSPLTFGQGTKLEIK

SEQ ID NO: 383 - protein, 108 aa, Artificial Sequence
  Synthetic peptide
DIQLTQSPSSLSASVGDRVTMTCTASSSVSSTYFHWYQQKPGKAPKLWIYSTSNLASGVPSRFSGSGSGTDYTLTISSMQPEDAATYYCHQYHRSPLTFGQGTKLEIK

SEQ ID NO: 384 - protein, 117 aa, Artificial Sequence
  Synthetic peptide
EVQLLESGGGLVQPGGSLRLSCAASGFTFSNYWMNWVRQAPGKGLEWVSQIRLKSDNYATHYADSVKGRFTISRDNSKNTLYLQMNSLRAEDTAVYYCAKGPPSGCWGQGTLVTVSS

SEQ ID NO: 385 - protein, 117 aa, Artificial Sequence
  Synthetic peptide
EVQLLESGGGLVQPGGSMRLSCAASGFTFSNYWMNWVRQAPGKGLEWVAQIRLKSDNYATHYADSVKGRFTISRDDSKNTVYLQMNSLRAEDTGVYYCNDGPPSGCWGQGTLLTVSS

SEQ ID NO: 386 - protein, 117 aa, Artificial Sequence
  Synthetic peptide
EVQLLESGGGLVQPGGSMRLSCAASGFTFSNYWMNWVRQAPGKGLEWVAQIRLKSDNYATHYADSVKGRFTISRDDSKNTVYLQMNSLRAEDTGVYYCNDGPPSGYWGQGTLLTVSS

SEQ ID NO: 387 - protein, 117 aa, Artificial Sequence
  Synthetic peptide
EVQLLESGGGLVQPGGSMRLSCAASGFTFSNYWMNWVRQAPGKGLEWVAQIRLKSDNYATHYADSVKGRFTISRDDSKNTVYLQMNSLRAEDTGVYYCNDGPPSGSWGQGTLLTVSS

SEQ ID NO: 388 - protein, 107 aa, Artificial Sequence
  Synthetic peptide
DIQMTQSPSSLSASVGDRVTITCRISENIYSYLAWYQQKPGKAPKLLIYNAKILVEGVPSRFSGSGSGTDFTLTISSLQPEDFATYYCQHHYTVPWTFGQGTKLEIK

SEQ ID NO: 389 - protein, 107 aa, Artificial Sequence
  Synthetic peptide
DIQMTQSPSSLSASVGDRVTITCRISENIYSYLAWYQQKPGKAPKLLVYNAKILVEGVPSRFSGSGSGTDFTLTISSLQPEDFGTYYCQHHYTVPWTFGQGTKLEIK

SEQ ID NO: 390 - protein, 107 aa, Artificial Sequence
  Synthetic peptide
DIQMTQSPSSLSASVGDRVTITCRISENIYSYLAWYQQKPGKAPKLLVYNAKSLVEGVPSRFSGSGSGTDFTLTISSLQPEDFGTYYCQHHYTVPWTFGQGTKLEIK

SEQ ID NO: 391 - protein, 117 aa, Artificial Sequence
  Synthetic peptide
QVQLVQSGAEVKKPGASVKVSCKASGYTFTSYTMHWVRQAPGQGLEWMGYINPSSTYTHYAQKFQGRVTMTRDTSTSTVYMELSSLRSEDTAVYYCARGELGGFAYWGQGTLVTVSS

SEQ ID NO: 392 - protein, 117 aa, Artificial Sequence
  Synthetic peptide
QVQLVQSGAEVKKPGASVKVSCKASGYTFTSYTMHWVRQAPGQGLEWMGYINPSSTYTHYAQKFQGRVTMTADTSTSTVYMELSSLRSEDTAVYYCSRGELGGFAYWGQGTLVTVSS

SEQ ID NO: 393 - protein, 117 aa, Artificial Sequence
  Synthetic peptide
QVQLVQSGAEVKKPGASVKMSCKASGYTFTSYTMHWIRQAPGQGLEWIGYINPSSTYTHYAQKFQGRATLTADTSTSTAYMELSSLRSEDTAVYYCSRGELGGFAYWGQGTLVTVSS

SEQ ID NO: 394 - protein, 117 aa, Artificial Sequence
  Synthetic peptide
QVQLVQSGAEVKKPGASVKMSCKASGYTFTSYTMHWIRQAPGQGQEWIGYINPSSTYTHYAQKFQGRATLTADTSTSTAYMELSSLRSEDTAVYYCSRGELGGFAYWGQGTLVTVSS

SEQ ID NO: 395 - protein, 117 aa, Artificial Sequence
  Synthetic peptide
QVQLVQSGAEVKKPGASVKMSCKASGYTFTSYTMHWIRQAPGQGLEWIGYINPSSTYTHYAQKFQGRATLTADKSTSTAYMELSSLRSEDTAVYYCSRGELGGFAYWGQGTLVTVSS

SEQ ID NO: 396 - protein, 117 aa, Artificial Sequence
  Synthetic peptide
QVQLVQSGAEVKKPGASVKMSCKASGYTFTSYTMHWIRQAPGQGQEWIGYINPSSTYTHYAQKFQGRATLTADKSTSTAYMELSSLRSEDTAVYYCSRGELGGFAYWGQGTLVTVSS

SEQ ID NO: 397 - protein, 112 aa, Artificial Sequence
  Synthetic peptide
DVVMTQSPLSLPVTLGQPASISCRSSQSLVHSDGNTYLNWFQQRPGQSPRRLIYKVSNRFSGVPDRFSGSGSGTDFTLKISRVEAEDVGVYYCSQSTHVPYTFGQGTKLEIK

SEQ ID NO: 398 - protein, 112 aa, Artificial Sequence
  Synthetic peptide
DVVMTQSPLSLPVTLGQPASISCRSSQSLVHSDGNTYLNWYQQRPGQSPRLLIYKVSNRFSGVPDRFSGSGSGTDFTLKISRVEAEDVGVYYCSQSTHVPYTFGQGTKLEIK

SEQ ID NO: 399 - protein, 112 aa, Artificial Sequence
  Synthetic peptide
DVVMTQSPLSLPVTLGQPASISCRSSQSLVHSEGNTYLNWYQQRPGQSPRLLIYKVSNRFSGVPDRFSGSGSGTDFTLKISRVEAEDVGVYYCSQSTHVPYTFGQGTKLEIK

SEQ ID NO: 400 - protein, 112 aa, Artificial Sequence
  Synthetic peptide
DVVMTQSPLSLPVTLGQPASISCRSSQSLVHSSGNTYLNWYQQRPGQSPRLLIYKVSNRFSGVPDRFSGSGSGTDFTLKISRVEAEDVGVYYCSQSTHVPYTFGQGTKLEIK

SEQ ID NO: 401 - protein, 112 aa, Artificial Sequence
  Synthetic peptide
DVVMTQSPLSLPVTLGQPASISCRSSQSLVHSEGSTYLNWYQQRPGQSPRLLIYKVSNRFSGVPDRFSGSGSGTDFTLKISRVEAEDVGVYYCSQSTHVPYTFGQGTKLEIK

SEQ ID NO: 402 - protein, 112 aa, Artificial Sequence
  Synthetic peptide
DVVMTQSPLSLPVTLGQPASISCRSSQSLVHSSGSTYLNWYQQRPGQSPRLLIYKVSNRFSGVPDRFSGSGSGTDFTLKISRVEAEDVGVYYCSQSTHVPYTFGQGTKLEIK

SEQ ID NO: 403 - protein, 117 aa, Artificial Sequence
  Synthetic peptide
QVQLVQSGAEVKKPGASVKVSCKASGYRFTDYNMHWVRQAPGQGLEWMGYINPNNGGTNYAQKFQGRVTMTRDTSTSTVYMELSSLRSEDTAVYYCARDYLYFFDCWGQGTLVTVSS

SEQ ID NO: 404 - protein, 117 aa, Artificial Sequence
  Synthetic peptide
QVQLVQSGAEVKKPGASVKVSCKASGYRFTDYNMHWVRQAPGQGLEWMGYINPNNGGTNYAQKFQGRVTMTVDTSTSTVYMELSSLRSEDTAVYYCARDYLYFFDCWGQGTLVTVSS

SEQ ID NO: 405 - protein, 117 aa, Artificial Sequence
  Synthetic peptide
QVQLVQSGAEVKKPGASVKMSCKASGYRFTDYNMHWVRQAPGQGLEWIGYINPNNGGTNYAQKFQGRATLTVDTSTSTAYMELSSLRSEDTAVYYCARDYLYFFDCWGQGTLLTVSS

SEQ ID NO: 406 - protein, 117 aa, Artificial Sequence
  Synthetic peptide
QVQLVQSGAEVKKPGASVKMSCKASGYRFTDYNMHWVRQAPGQGLEWIGYINPNNGGTNYAQKFQGRATLTVDKSTSTAYMELSSLRSEDTAVYYCARDYLYFFDCWGQGTLLTVSS

SEQ ID NO: 407 - protein, 117 aa, Artificial Sequence
  Synthetic peptide
QVQLVQSGAEVKKPGASVKMSCKASGYRFTDYNMHWVRQAPGQGLEWIGYINPNNGGTNYAQKFQGRATLTVNKSTSTAYMELSSLRSEDTAVYYCARDYLYFFDCWGQGTLLTVSS

SEQ ID NO: 408 - protein, 117 aa, Artificial Sequence
  Synthetic peptide
QVQLVQSGAEVKKPGASVKMSCKASGYRFTDYNMHWVRQAPGQGLEWIGYINPNNGGTNYAQKFQGRATLTVNTSTSTAYMELSSLRSEDTAVYYCARDYLYFFDCWGQGTLLTVSS

SEQ ID NO: 409 - protein, 107 aa, Artificial Sequence
  Synthetic peptide
DIQMTQSPSSLSASVGDRVTITCLASQTIGTWLAWYQQKPGKAPKLLIYAAASLADGVPSRFSGSGSGTDFTLTISSLQPEDFATYYCQQLYSIPRTFGQGTKLEIK

SEQ ID NO: 410 - protein, 107 aa, Artificial Sequence
  Synthetic peptide
DIQMTQSPSSLSASVGDRVTITCLASQTIGTWLAWYQQKPGKAPKLLIYAAASLADGVPSRFSGSGSGTDFTFTISSLQPEDFVTYYCQQLYSIPRTFGQGTKLEIK

SEQ ID NO: 411 - protein, 107 aa, Artificial Sequence
  Synthetic peptide
DIQMTQSPSSLSASVGDRVTITCRASQTIGTWLAWYQQKPGKAPKLLIYAAASLADGVPSRFSGSGSGTDFTFTISSLQPEDFVTYYCQQLYSIPRTFGQGTKLEIK

SEQ ID NO: 412 - protein, 118 aa, Artificial Sequence
  Synthetic peptide
EVQLVESGGGLVQPGGSLRLSCAASGFTFSSFGMHWVRQAPGKGLEWVSYISSDSRTIYYADSVKGRFTISRDNAKNSLYLQMNSLRAEDTAVYYCARDYGRTYEAYWGQGTLVTVSS

SEQ ID NO: 413 - protein, 118 aa, Artificial Sequence
  Synthetic peptide
EVQLVESGGGLVQPGGSLRLSCAASGFTFSSFGMHWVRQAPGKGLEWVAYISSDSRTIYYADSVKGRFTISRDNAKNSLYLQMNSLRAEDTAVYYCARDYGRTYEAYWGQGTLVTVSS

SEQ ID NO: 414 - protein, 111 aa, Artificial Sequence
  Synthetic peptide
DIVMTQSPDSLAVSLGERATINCRASKSVSTSGYSYIHWYQQKPGQPPKLLIYLASNLESGVPDRFSGSGSGTDFTLTISSLQAEDVAVYYCQHSRELPLTFGQGTKLEIK

SEQ ID NO: 415 - protein, 111 aa, Artificial Sequence
  Synthetic peptide
DIVLTQSPDSLAVSLGERATINCRASKSVSTSGYSYIHWYQQKPGQPPKLLIYLASNLESGVPDRFSGSGSGTDFTLTISSVQAEDVAVYYCQHSRELPLTFGQGTKLELK

SEQ ID NO: 416 - protein, 121 aa, Artificial Sequence
  Synthetic peptide
QVQLVQSGAEVKKPGASVKVSCKASGYSFTGYNMNWVRQAPGQGLEWMGNIDPYYGGSTYAQKFQGRVTMTRDTSTSTVYMELSSLRSEDTAVYYCARERSGYVFSAMDYWGQGTLVTVSS

SEQ ID NO: 417 - protein, 121 aa, Artificial Sequence
  Synthetic peptide
QVQLVQSGAEVKKPGASVKVSCKASGYSFTGYNMNWVRQAPGQGLEWMGNIDPYYGGSTYAQKFQGRVTMTVDTSTSTVYMELSSLRSEDTAVYYCARERSGYVFSAMDYWGQGTLVTVSS

SEQ ID NO: 418 - protein, 121 aa, Artificial Sequence
  Synthetic peptide
QVQLVQSGAEVKKPGASVKISCKASGYSFTGYNMNWVRQAPGQGLEWIGNIDPYYGGSTYAQKFQGRATLTVDTSTSTAYMELSSLRSEDTAVYYCARERSGYVFSAMDYWGQGTLVTVSS

SEQ ID NO: 419 - protein, 121 aa, Artificial Sequence
  Synthetic peptide
QVQLVQSGAEVKKPGASVKISCKASGYSFTGYNMNWVRQAPGQGLEWIGNIDPYYGGSTYAQKFQGRATLTVDKSTSTAYMELSSLRSEDTAVYYCARERSGYVFSAMDYWGQGTLVTVSS

SEQ ID NO: 420 - protein, 112 aa, Artificial Sequence
  Synthetic peptide
DIVMTQSPDSLAVSLGERATINCKSSQSVLFSSNQKNYLAWYQQKPGQPPKLLIYWASTRESGVPDRFSGSGSGTDFTLTISSLQAEDVAVYYCHQYLSSRTFGQGTKLEIK

SEQ ID NO: 421 - protein, 112 aa, Artificial Sequence
  Synthetic peptide
DIVMTQSPDSLAVSLGERVTMNCKSSQSVLFSSNQKNYLAWYQQKPGQPPKLLIYWASTRESGVPDRFSGSGSGTDFTLTISSVQAEDVAVYYCHQYLSSRTFGQGTKLEIK

SEQ ID NO: 422 - protein, 117 aa, Artificial Sequence
  Synthetic peptide
EVQLLESGGGLVQPGGSMRLSCAASGFTFSNYWMNWVRQAPGKGLEWVAQIRLKSDNYATHYADSVKGRFTISRDDSKNTVYLQMNSLRAEDTGVYYCNDGPPSGAWGQGTLLTVSS

SEQ ID NO: 423 - protein, 117 aa, Artificial Sequence
  Synthetic peptide
QVQLVQSGAEVKKPGASVKVSCKASGYTFTSYTMHWVRQAPGQGLEWMGYINPSSTYTHYIKKFKDRVTMTADTSTSTVYMELSSLRSEDTAVYYCSRGELGGFAYWGQGTLVTVSS

SEQ ID NO: 424 - protein, 117 aa, Artificial Sequence
  Synthetic peptide
QVQLVQSGAEVKKPGASVKMSCKASGYTFTSYTMHWIRQAPGQGLEWIGYINPSSTYTHYIKKFKDRATLTADTSTSTAYMELSSLRSEDTAVYYCSRGELGGFAYWGQGTLVTVSS

SEQ ID NO: 425 - protein, 117 aa, Artificial Sequence
  Synthetic peptide
QVQLVQSGAEVKKPGASVKMSCKASGYTFTSYTMHWIRQAPGQGQEWIGYINPSSTYTHYIKKFKDRATLTADTSTSTAYMELSSLRSEDTAVYYCSRGELGGFAYWGQGTLVTVSS

SEQ ID NO: 426 - protein, 117 aa, Artificial Sequence
  Synthetic peptide
QVQLVQSGAEVKKPGASVKMSCKASGYTFTSYTMHWIRQAPGQGLEWIGYINPSSTYTHYIKKFKDRATLTADKSTSTAYMELSSLRSEDTAVYYCSRGELGGFAYWGQGTLVTVSS

SEQ ID NO: 427 - protein, 117 aa, Artificial Sequence
  Synthetic peptide
QVQLVQSGAEVKKPGASVKMSCKASGYTFTSYTMHWIRQAPGQGQEWIGYINPSSTYTHYIKKFKDRATLTADKSTSTAYMELSSLRSEDTAVYYCSRGELGGFAYWGQGTLVTVSS

SEQ ID NO: 428 - protein, 116 aa, Artificial Sequence
  Synthetic peptide
  misc_feature (5)..(5): Xaa can be any naturally occurring amino acid
  misc_feature (8)..(8): Xaa can be any naturally occurring amino acid
  misc_feature (11)..(13): Xaa can be any naturally occurring amino acid
  misc_feature (20)..(20): Xaa can be any naturally occurring amino acid
  misc_feature (31)..(31): Xaa can be any naturally occurring amino acid
  misc_feature (33)..(33): Xaa can be any naturally occurring amino acid
  misc_feature (35)..(35): Xaa can be any naturally occurring amino acid
  misc_feature (38)..(38): Xaa can be any naturally occurring amino acid
  misc_feature (40)..(40): Xaa can be any naturally occurring amino acid
  misc_feature (48)..(48): Xaa can be any naturally occurring amino acid
  misc_feature (50)..(50): Xaa can be any naturally occurring amino acid
  misc_feature (55)..(55): Xaa can be any naturally occurring amino acid
  misc_feature (57)..(57): Xaa can be any naturally occurring amino acid
  misc_feature (59)..(59): Xaa can be any naturally occurring amino acid
  misc_feature (61)..(61): Xaa can be any naturally occurring amino acid
  misc_feature (65)..(68): Xaa can be any naturally occurring amino acid
  misc_feature (70)..(70): Xaa can be any naturally occurring amino acid
  misc_feature (72)..(72): Xaa can be any naturally occurring amino acid
  misc_feature (74)..(76): Xaa can be any naturally occurring amino acid
  misc_feature (79)..(80): Xaa can be any naturally occurring amino acid
  misc_feature (82)..(82): Xaa can be any naturally occurring amino acid
  misc_feature (87)..(87): Xaa can be any naturally occurring amino acid
  misc_feature (90)..(91): Xaa can be any naturally occurring amino acid
  misc_feature (98)..(98): Xaa can be any naturally occurring amino acid
  misc_feature (101)..(101): Xaa can be any naturally occurring amino acid
  misc_feature (116)..(116): Xaa can be any naturally occurring amino acid
QVQLXQSXAEXXXPGASVKXSCKASGYTFTXYXMXWVXQXPGQGLEWXGXINPSXGXTXYXQKFXXXXTXTXDXSXSTXXMXLSSLXSEXXAVYYCAXGDXYVAYWGQGTLVTVSX

SEQ ID NO: 429 - protein, 116 aa, Artificial Sequence
  Synthetic peptide
  misc_feature (20)..(20): Xaa can be any naturally occurring amino acid
  misc_feature (31)..(31): Xaa can be any naturally occurring amino acid
  misc_feature (35)..(35): Xaa can be any naturally occurring amino acid
  misc_feature (48)..(48): Xaa can be any naturally occurring amino acid
  misc_feature (50)..(50): Xaa can be any naturally occurring amino acid
  misc_feature (59)..(59): Xaa can be any naturally occurring amino acid
  misc_feature (67)..(67): Xaa can be any naturally occurring amino acid
  misc_feature (70)..(70): Xaa can be any naturally occurring amino acid
  misc_feature (74)..(74): Xaa can be any naturally occurring amino acid
  misc_feature (79)..(79): Xaa can be any naturally occurring amino acid
  misc_feature (98)..(98): Xaa can be any naturally occurring amino acid
  misc_feature (101)..(101): Xaa can be any naturally occurring amino acid
QVQLVQSGAEVKKPGASVKXSCKASGYTFTXYTMXWVRQAPGQGLEWXGXINPSSGYTXYAQKFQGXVTXTADXSTSTXYMELSSLRSEDTAVYYCAXGDXYVAYWGQGTLVTVSS

SEQ ID NO: 430 - protein, 108 aa, Artificial Sequence
  Synthetic peptide
  misc_feature (1)..(1): Xaa can be any naturally occurring amino acid
  misc_feature (3)..(4): Xaa can be any naturally occurring amino acid
  misc_feature (9)..(11): Xaa can be any naturally occurring amino acid
  misc_feature (15)..(15): Xaa can be any naturally occurring amino acid
  misc_feature (17)..(17): Xaa can be any naturally occurring amino acid
  misc_feature (21)..(21): Xaa can be any naturally occurring amino acid
  misc_feature (24)..(24): Xaa can be any naturally occurring amino acid
  misc_feature (27)..(27): Xaa can be any naturally occurring amino acid
  misc_feature (29)..(29): Xaa can be any naturally occurring amino acid
  misc_feature (32)..(32): Xaa can be any naturally occurring amino acid
  misc_feature (34)..(35): Xaa can be any naturally occurring amino acid
  misc_feature (43)..(44): Xaa can be any naturally occurring amino acid
  misc_feature (48)..(48): Xaa can be any naturally occurring amino acid
  misc_feature (51)..(56): Xaa can be any naturally occurring amino acid
  misc_feature (61)..(61): Xaa can be any naturally occurring amino acid
  misc_feature (67)..(67): Xaa can be any naturally occurring amino acid
  misc_feature (71)..(73): Xaa can be any naturally occurring amino acid
  misc_feature (79)..(81): Xaa can be any naturally occurring amino acid
  misc_feature (84)..(84): Xaa can be any naturally occurring amino acid
  misc_feature (90)..(91): Xaa can be any naturally occurring amino acid
  misc_feature (93)..(96): Xaa can be any naturally occurring amino acid
  misc_feature (101)..(101): Xaa can be any naturally occurring amino acid
  misc_feature (107)..(107): Xaa can be any naturally occurring amino acid
XIXXTQSPXXXSASXGXRVTXTCXASXSXSSXYXXWYQQKPGXXPKLXIYXXXXXXSGVPXRFSGSXSGTXXXLTISSXXXEDXATYYCXXYXXXXLTFGXGTKLEXK

SEQ ID NO: 431 - protein, 108 aa, Artificial Sequence
  Synthetic peptide
  misc_feature (4)..(4): Xaa can be any naturally occurring amino acid
  misc_feature (21)..(21): Xaa can be any naturally occurring amino acid
  misc_feature (32)..(32): Xaa can be any naturally occurring amino acid
  misc_feature (34)..(34): Xaa can be any naturally occurring amino acid
  misc_feature (48)..(48): Xaa can be any naturally occurring amino acid
  misc_feature (51)..(51): Xaa can be any naturally occurring amino acid
  misc_feature (53)..(53): Xaa can be any naturally occurring amino acid
  misc_feature (61)..(61): Xaa can be any naturally occurring amino acid
  misc_feature (67)..(67): Xaa can be any naturally occurring amino acid
  misc_feature (79)..(79): Xaa can be any naturally occurring amino acid
  misc_feature (84)..(84): Xaa can be any naturally occurring amino acid
  misc_feature (91)..(91): Xaa can be any naturally occurring amino acid
  misc_feature (93)..(93): Xaa can be any naturally occurring amino acid
DIQXTQSPSSLSASVGDRVTXTCTASSSVSSXYXHWYQQKPGKAPKLXIYXTXNLASGVPXRFSGSXSGTDYTLTISSXQPEDXATYYCHXYXRSPLTFGQGTKLEIK

SEQ ID NO: 432 - protein, 117 aa, Artificial Sequence
  Synthetic peptide
  misc_feature (3)..(3): Xaa can be any naturally occurring amino acid
  misc_feature (5)..(5): Xaa can be any naturally occurring amino acid
  misc_feature (18)..(19): Xaa can be any naturally occurring amino acid
  misc_feature (23)..(23): Xaa can be any naturally occurring amino acid
  misc_feature (31)..(31): Xaa can be any naturally occurring amino acid
  misc_feature (33)..(33): Xaa can be any naturally occurring amino acid
  misc_feature (35)..(35): Xaa can be any naturally occurring amino acid
  misc_feature (40)..(40): Xaa can be any naturally occurring amino acid
  misc_feature (42)..(42): Xaa can be any naturally occurring amino acid
  misc_feature (49)..(50): Xaa can be any naturally occurring amino acid
  misc_feature (52)..(59): Xaa can be any naturally occurring amino acid
  misc_feature (61)..(61): Xaa can be any naturally occurring amino acid
  misc_feature (64)..(64): Xaa can be any naturally occurring amino acid
  misc_feature (76)..(76): Xaa can be any naturally occurring amino acid
  misc_feature (79)..(81): Xaa can be any naturally occurring amino acid
  misc_feature (87)..(87): Xaa can be any naturally occurring amino acid
  misc_feature (94)..(95): Xaa can be any naturally occurring amino acid
  misc_feature (99)..(99): Xaa can be any naturally occurring amino acid
  misc_feature (106)..(106): Xaa can be any naturally occurring amino acid
  misc_feature (112)..(112): Xaa can be any naturally occurring amino acid
  misc_feature (114)..(114): Xaa can be any naturally occurring amino acid
EVXLXESGGGLVQPGGSXXLSCXASGFTFSXYXMXWVRQXPXKGLEWVXXIXXXXXXXXTXYAXSVKGRFTISRDXSKXXXYLQMNXLRAEDTXXYYCXDGPPSGXWGQGTXLXVSS

SEQ ID NO: 433 - protein, 117 aa, Artificial Sequence
  Synthetic peptide
  misc_feature (31)..(31): Xaa can be any naturally occurring amino acid
  misc_feature (35)..(35): Xaa can be any naturally occurring amino acid
  misc_feature (50)..(50): Xaa can be any naturally occurring amino acid
  misc_feature (55)..(55): Xaa can be any naturally occurring amino acid
  misc_feature (79)..(79): Xaa can be any naturally occurring amino acid
  misc_feature (99)..(99): Xaa can be any naturally occurring amino acid
  misc_feature (106)..(106): Xaa can be any naturally occurring amino acid
EVQLLESGGGLVQPGGSMRLSCAASGFTFSXYWMXWVRQAPGKGLEWVAXIRLKXDNYATHYADSVKGRFTISRDDSKXTVYLQMNSLRAEDTGVYYCXDGPPSGXWGQGTLLTVSS

SEQ ID NO: 434 - protein, 107 aa, Artificial Sequence
  Synthetic peptide
  misc_feature (9)..(9): Xaa can be any naturally occurring amino acid
  misc_feature (17)..(18): Xaa can be any naturally occurring amino acid
  misc_feature (25)..(25): Xaa can be any naturally occurring amino acid
  misc_feature (27)..(28): Xaa can be any naturally occurring amino acid
  misc_feature (30)..(30): Xaa can be any naturally occurring amino acid
  misc_feature (34)..(34): Xaa can be any naturally occurring amino acid
  misc_feature (40)..(40): Xaa can be any naturally occurring amino acid
  misc_feature (43)..(43): Xaa can be any naturally occurring amino acid
  misc_feature (45)..(45): Xaa can be any naturally occurring amino acid
  misc_feature (48)..(48): Xaa can be any naturally occurring amino acid
  misc_feature (50)..(50): Xaa can be any naturally occurring amino acid
  misc_feature (52)..(53): Xaa can be any naturally occurring amino acid
  misc_feature (55)..(56): Xaa can be any naturally occurring amino acid
  misc_feature (70)..(70): Xaa can be any naturally occurring amino acid
  misc_feature (72)..(72): Xaa can be any naturally occurring amino acid
  misc_feature (74)..(74): Xaa can be any naturally occurring amino acid
  misc_feature (76)..(76): Xaa can be any naturally occurring amino acid
  misc_feature (84)..(85): Xaa can be any naturally occurring amino acid
  misc_feature (90)..(91): Xaa can be any naturally occurring amino acid
  misc_feature (93)..(94): Xaa can be any naturally occurring amino acid
  misc_feature (97)..(97): Xaa can be any naturally occurring amino acid
  misc_feature (100)..(100): Xaa can be any naturally occurring amino acid
DIQMTQSPXSLSASVGXXVTITCRXSXXIXSYLXWYQQKXGKXPXLLXYXAXXLXXGVPSRFSGSGSGTXFXLXIXSLQPEDFXXYYCQXXYXXPWXFGXGTKLEIK

SEQ ID NO: 435 - protein, 107 aa, Artificial Sequence
  Synthetic peptide
  misc_feature (25)..(25): Xaa can be any naturally occurring amino acid
  misc_feature (34)..(34): Xaa can be any naturally occurring amino acid
  misc_feature (48)..(48): Xaa can be any naturally occurring amino acid
  misc_feature (53)..(53): Xaa can be any naturally occurring amino acid
  misc_feature (55)..(55): Xaa can be any naturally occurring amino acid
  misc_feature (84)..(85): Xaa can be any naturally occurring amino acid
  misc_feature (90)..(90): Xaa can be any naturally occurring amino acid
  misc_feature (93)..(93): Xaa can be any naturally occurring amino acid
DIQMTQSPSSLSASVGDRVTITCRXSENIYSYLXWYQQKPGKAPKLLXYNAKXLXEGVPSRFSGSGSGTDFTLTISSLQPEDFXXYYCQXHYXVPWTFGQGTKLEIK

SEQ ID NO: 436 - protein, 117 aa, Artificial Sequence
  Synthetic peptide
  misc_feature (5)..(5): Xaa can be any naturally occurring amino acid
  misc_feature (11)..(13): Xaa can be any naturally occurring amino acid
  misc_feature (20)..(20): Xaa can be any naturally occurring amino acid
  misc_feature (29)..(29): Xaa can be any naturally occurring amino acid
  misc_feature (31)..(31): Xaa can be any naturally occurring amino acid
  misc_feature (33)..(33): Xaa can be any naturally occurring amino acid
  misc_feature (37)..(38): Xaa can be any naturally occurring amino acid
  misc_feature (40)..(40): Xaa can be any naturally occurring amino acid
  misc_feature (45)..(45): Xaa can be any naturally occurring amino acid
  misc_feature (48)..(48): Xaa can be any naturally occurring amino acid
  misc_feature (50)..(50): Xaa can be any naturally occurring amino acid
  misc_feature (55)..(57): Xaa can be any naturally occurring amino acid
  misc_feature (59)..(59): Xaa can be any naturally occurring amino acid
  misc_feature (61)..(62): Xaa can be any naturally occurring amino acid
  misc_feature (65)..(68): Xaa can be any naturally occurring amino acid
  misc_feature (70)..(70): Xaa can be any naturally occurring amino acid
  misc_feature (72)..(72): Xaa can be any naturally occurring amino acid
  misc_feature (74)..(74): Xaa can be any naturally occurring amino acid
  misc_feature (76)..(76): Xaa can be any naturally occurring amino acid
  misc_feature (79)..(79): Xaa can be any naturally occurring amino acid
  misc_feature (82)..(82): Xaa can be any naturally occurring amino acid
  misc_feature (84)..(84): Xaa can be any naturally occurring amino acid
  misc_feature (87)..(87): Xaa can be any naturally occurring amino acid
  misc_feature (91)..(91): Xaa can be any naturally occurring amino acid
  misc_feature (97)..(97): Xaa can be any naturally occurring amino acid
  misc_feature (101)..(101): Xaa can be any naturally occurring amino acid
  misc_feature (117)..(117): Xaa can be any naturally occurring amino acid
QVQLXQSGAEXXXPGASVKXSCKASGYTXTXYXMHWXXQXPGQGXEWXGXINPSXXXTXYXXKFXXXXTXTXDXSXSTXYMXLXSLXSEDXAVYYCXRGEXGGFAYWGQGTLVTVSX

SEQ ID NO: 437 - protein, 117 aa, Artificial Sequence
  Synthetic peptide
  misc_feature (20)..(20): Xaa can be any naturally occurring amino acid
  misc_feature (29)..(29): Xaa can be any naturally occurring amino acid
  misc_feature (31)..(31): Xaa can be any naturally occurring amino acid
  misc_feature (37)..(37): Xaa can be any naturally occurring amino acid
  misc_feature (45)..(45): Xaa can be any naturally occurring amino acid
  misc_feature (48)..(48): Xaa can be any naturally occurring amino acid
  misc_feature (56)..(56): Xaa can be any naturally occurring amino acid
  misc_feature (59)..(59): Xaa can be any naturally occurring amino acid
  misc_feature (61)..(62): Xaa can be any naturally occurring amino acid
  misc_feature (65)..(66): Xaa can be any naturally occurring amino acid
  misc_feature (68)..(68): Xaa can be any naturally occurring amino acid
  misc_feature (70)..(70): Xaa can be any naturally occurring amino acid
  misc_feature (74)..(74): Xaa can be any naturally occurring amino acid
  misc_feature (79)..(79): Xaa can be any naturally occurring amino acid
  misc_feature (84)..(84): Xaa can be any naturally occurring amino acid
  misc_feature (97)..(97): Xaa can be any naturally occurring amino acid
  misc_feature (101)..(101): Xaa can be any naturally occurring amino acid
QVQLVQSGAEVKKPGASVKXSCKASGYTXTXYTMHWXRQAPGQGXEWXGYINPSSXYTXYXXKFXXRXTXTADXSTSTXYMELXSLRSEDTAVYYCXRGEXGGFAYWGQGTLVTVSS

SEQ ID NO: 438 - protein, 112 aa, Artificial Sequence
  Synthetic peptide
  misc_feature (7)..(7): Xaa can be any naturally occurring amino acid
  misc_feature (14)..(14): Xaa can be any naturally occurring amino acid
  misc_feature (17)..(18): Xaa can be any naturally occurring amino acid
  misc_feature (31)..(31): Xaa can be any naturally occurring amino acid
  misc_feature (33)..(33): Xaa can be any naturally occurring amino acid
  misc_feature (39)..(39): Xaa can be any naturally occurring amino acid
  misc_feature (41)..(42): Xaa can be any naturally occurring amino acid
  misc_feature (44)..(44): Xaa can be any naturally occurring amino acid
  misc_feature (50)..(51): Xaa can be any naturally occurring amino acid
  misc_feature (55)..(55): Xaa can be any naturally occurring amino acid
  misc_feature (57)..(57): Xaa can be any naturally occurring amino acid
  misc_feature (81)..(81): Xaa can be any naturally occurring amino acid
  misc_feature (88)..(88): Xaa can be any naturally occurring amino acid
  misc_feature (92)..(92): Xaa can be any naturally occurring amino acid
  misc_feature (94)..(96): Xaa can be any naturally occurring amino acid
  misc_feature (99)..(100): Xaa can be any naturally occurring amino acid
  misc_feature (105)..(105): Xaa can be any naturally occurring amino acid
DVVMTQXPLSLPVXLGXXASISCRSSQSLVXSXGNTYLXWXXQXPGQSPXXNPSXTXTHYSGVPDRFSGSGSGTDFTLKIXRVEAEDXGVYXCXXXTHXXYTFGXGTKLEIK

SEQ ID NO: 439 - protein, 112 aa, Artificial Sequence
  Synthetic peptide
  misc_feature (33)..(33): Xaa can be any naturally occurring amino acid
  misc_feature (39)..(39): Xaa can be any naturally occurring amino acid
  misc_feature (55)..(55): Xaa can be any naturally occurring amino acid
  misc_feature (57)..(57): Xaa can be any naturally occurring amino acid
  misc_feature (81)..(81): Xaa can be any naturally occurring amino acid
  misc_feature (95)..(96): Xaa can be any naturally occurring amino acid
DVVMTQSPLSLPVTLGQPASISCRSSQSLVHSXGNTYLXWYQQRPGQSPRLLIYXVXNRFSGVPDRFSGSGSGTDFTLKIXRVEAEDVGVYYCSXXTHVPYTFGQGTKLEIK

SEQ ID NO: 440 - protein, 120 aa, Artificial Sequence
  Synthetic peptide
  misc_feature (5)..(5): Xaa can be any naturally occurring amino acid
  misc_feature (9)..(9): Xaa can be any naturally occurring amino acid
  misc_feature (11)..(12): Xaa can be any naturally occurring amino acid
  misc_feature (20)..(20): Xaa can be any naturally occurring amino acid
  misc_feature (38)..(38): Xaa can be any naturally occurring amino acid
  misc_feature (40)..(41): Xaa can be any naturally occurring amino acid
  misc_feature (43)..(44): Xaa can be any naturally occurring amino acid
  misc_feature (48)..(48): Xaa can be any naturally occurring amino acid
  misc_feature (61)..(61): Xaa can be any naturally occurring amino acid
  misc_feature (65)..(65): Xaa can be any naturally occurring amino acid
  misc_feature (67)..(68): Xaa can be any naturally occurring amino acid
  misc_feature (70)..(70): Xaa can be any naturally occurring amino acid
  misc_feature (72)..(72): Xaa can be any naturally occurring amino acid
  misc_feature (74)..(74): Xaa can be any naturally occurring amino acid
  misc_feature (76)..(76): Xaa can be any naturally occurring amino acid
  misc_feature (79)..(79): Xaa can be any naturally occurring amino acid
  misc_feature (82)..(82): Xaa can be any naturally occurring amino acid
  misc_feature (84)..(84): Xaa can be any naturally occurring amino acid
  misc_feature (87)..(87): Xaa can be any naturally occurring amino acid
  misc_feature (91)..(91): Xaa can be any naturally occurring amino acid
  misc_feature (116)..(116): Xaa can be any naturally occurring amino acid
QVQLXQSGXEXXKPGASVKXSCKASGYSFTGYNMNWVXQXXGXXLEWXGNIDPYYGGSTYXQKFXGXXTXTXDXSXSTXYMXLXSLXSEDXAVYYCARERSGYVFSAMDYWGQGTXVTVS

SEQ ID NO: 441 - protein, 120 aa, Artificial Sequence
  Synthetic peptide
  misc_feature (20)..(20): Xaa can be any naturally occurring amino acid
  misc_feature (48)..(48): Xaa can be any naturally occurring amino acid
  misc_feature (68)..(68): Xaa can be any naturally occurring amino acid
  misc_feature (70)..(70): Xaa can be any naturally occurring amino acid
  misc_feature (79)..(79): Xaa can be any naturally occurring amino acid
QVQLVQSGAEVKKPGASVKXSCKASGYSFTGYNMNWVRQAPGQGLEWXGNIDPYYGGSTYAQKFQGRXTXTRDTSTSTXYMELSSLRSEDTAVYYCARERSGYVFSAMDYWGQGTLVTVS

SEQ ID NO: 442 - protein, 112 aa, Artificial Sequence
  Synthetic peptide
  misc_feature (1)..(1): Xaa can be any naturally occurring amino acid
  misc_feature (3)..(3): Xaa can be any naturally occurring amino acid
  misc_feature (9)..(9): Xaa can be any naturally occurring amino acid
  misc_feature (15)..(15): Xaa can be any naturally occurring amino acid
  misc_feature (18)..(19): Xaa can be any naturally occurring amino acid
  misc_feature (21)..(22): Xaa can be any naturally occurring amino acid
  misc_feature (49)..(49): Xaa can be any naturally occurring amino acid
  misc_feature (51)..(51): Xaa can be any naturally occurring amino acid
  misc_feature (69)..(69): Xaa can be any naturally occurring amino acid
  misc_feature (78)..(78): Xaa can be any naturally occurring amino acid
  misc_feature (84)..(84): Xaa can be any naturally occurring amino acid
  misc_feature (93)..(93): Xaa can be any naturally occurring amino acid
  misc_feature (105)..(105): Xaa can be any naturally occurring amino acid
  misc_feature (111)..(111): Xaa can be any naturally occurring amino acid
XIXMTQSPXSLAVSXGEXXTXXCKSSQSVLFSSNQKNYLAWYQQKPGQXPXLLIYWASTRESGVPDRFXGSGSGTDFXLTISSXQAEDVAVYXCHQYLSSRTFGXGTKLEXK

SEQ ID NO: 443 - protein, 112 aa, Artificial Sequence
  Synthetic peptide
  misc_feature (19)..(19): Xaa can be any naturally occurring amino acid
  misc_feature (21)..(21): Xaa can be any naturally occurring amino acid
  misc_feature (84)..(84): Xaa can be any naturally occurring amino acid
DIVMTQSPDSLAVSLGERXTXNCKSSQSVLFSSNQKNYLAWYQQKPGQPPKLLIYWASTRESGVPDRFSGSGSGTDFTLTISSXQAEDVAVYYCHQYLSSRTFGQGTKLEIK

SEQ ID NO: 444 - protein, 117 aa, Artificial Sequence
  Synthetic peptide
  misc_feature (1)..(1): Xaa can be any naturally occurring amino acid
  misc_feature (5)..(5): Xaa can be any naturally occurring amino acid
  misc_feature (9)..(9): Xaa can be any naturally occurring amino acid
  misc_feature (11)..(12): Xaa can be any naturally occurring amino acid
  misc_feature (20)..(20): Xaa can be any naturally occurring amino acid
  misc_feature (38)..(38): Xaa can be any naturally occurring amino acid
  misc_feature (40)..(41): Xaa can be any naturally occurring amino acid
  misc_feature (43)..(44): Xaa can be any naturally occurring amino acid
  misc_feature (48)..(48): Xaa can be any naturally occurring amino acid
  misc_feature (61)..(61): Xaa can be any naturally occurring amino acid
  misc_feature (63)..(63): Xaa can be any naturally occurring amino acid
  misc_feature (65)..(65): Xaa can be any naturally occurring amino acid
  misc_feature (67)..(67): Xaa can be any naturally occurring amino acid
  misc_feature (69)..(70): Xaa can be any naturally occurring amino acid
  misc_feature (72)..(74): Xaa can be any naturally occurring amino acid
  misc_feature (76)..(76): Xaa can be any naturally occurring amino acid
  misc_feature (79)..(79): Xaa can be any naturally occurring amino acid
  misc_feature (84)..(84): Xaa can be any naturally occurring amino acid
  misc_feature (87)..(87): Xaa can be any naturally occurring amino acid
  misc_feature (91)..(91): Xaa can be any naturally occurring amino acid
  misc_feature (93)..(93): Xaa can be any naturally occurring amino acid
  misc_feature (112)..(113): Xaa can be any naturally occurring amino acid
XVQLXQSGXEXXKPGASVKXSCKASGYRFTDYNMHWVXQXXGXXLEWXGYINPNNGGTNYXQXFXGXVXXTXXXSXSTXYMELXSLXSEDXAXYYCARDYLYFFDCWGQGTXXTVSS

SEQ ID NO: 445 - protein, 107 aa, Artificial Sequence
  Synthetic peptide
  misc_feature (9)..(9): Xaa can be any naturally occurring amino acid
  misc_feature (11)..(11): Xaa can be any naturally occurring amino acid
  misc_feature (15)..(15): Xaa can be any naturally occurring amino acid
  misc_feature (17)..(18): Xaa can be any naturally occurring amino acid
  misc_feature (43)..(43): Xaa can be any naturally occurring amino acid
  misc_feature (45)..(45): Xaa can be any naturally occurring amino acid
  misc_feature (70)..(70): Xaa can be any naturally occurring amino acid
  misc_feature (72)..(74): Xaa can be any naturally occurring amino acid
  misc_feature (80)..(80): Xaa can be any naturally occurring amino acid
  misc_feature (84)..(85): Xaa can be any naturally occurring amino acid
  misc_feature (100)..(100): Xaa can be any naturally occurring amino acid
DIQMTQSPXSXSASXGXXVTITCLASQTIGTWLAWYQQKPGKXPXLLIYAAASLADGVPSRFSGSGSGTXFXXXISSLQXEDFXXYYCQQLYSIPRTFGXGTKLEIK

SEQ ID NO: 446 - protein, 107 aa, Artificial Sequence
  Synthetic peptide
  misc_feature (1)..(1): Xaa can be any naturally occurring amino acid
  misc_feature (15)..(15): Xaa can be any naturally occurring amino acid
  misc_feature (18)..(19): Xaa can be any naturally occurring amino acid
  misc_feature (42)..(42): Xaa can be any naturally occurring amino acid
  misc_feature (49)..(49): Xaa can be any naturally occurring amino acid
  misc_feature (63)..(63): Xaa can be any naturally occurring amino acid
  misc_feature (75)..(76): Xaa can be any naturally occurring amino acid
  misc_feature (78)..(78): Xaa can be any naturally occurring amino acid
  misc_feature (80)..(80): Xaa can be any naturally occurring amino acid
  misc_feature (84)..(84): Xaa can be any naturally occurring amino acid
  misc_feature (88)..(88): Xaa can be any naturally occurring amino acid
  misc_feature (93)..(93): Xaa can be any naturally occurring amino acid
XVQLVESGGGLVQPXGSXXLSCAASGFTFSSFGMHWVRQAPXKGLEWVXYISSDSRTIYYADXVKGRFTISRDNXXNXLXLQMXSLRXEDTAXYYCARDYGRTYEAY

SEQ ID NO: 447 - protein, 111 aa, Artificial Sequence
  Synthetic peptide
  misc_feature (4)..(4): Xaa can be any naturally occurring amino acid
  misc_feature (9)..(9): Xaa can be any naturally occurring amino acid
  misc_feature (17)..(17): Xaa can be any naturally occurring amino acid
  misc_feature (22)..(22): Xaa can be any naturally occurring amino acid
  misc_feature (64)..(64): Xaa can be any naturally occurring amino acid
  misc_feature (78)..(78): Xaa can be any naturally occurring amino acid
  misc_feature (80)..(84): Xaa can be any naturally occurring amino acid
  misc_feature (87)..(87): Xaa can be any naturally occurring amino acid
  misc_feature (89)..(89): Xaa can be any naturally occurring amino acid
  misc_feature (104)..(104): Xaa can be any naturally occurring amino acid
  misc_feature (110)..(110): Xaa can be any naturally occurring amino acid
DIVXTQSPXSLAVSLGXRATIXCRASKSVSTSGYSYIHWYQQKPGQPPKLLIYLASNLESGVPXRFSGSGSGTDFTLXIXXXXXEDXAXYYCQHSRELPLTFGXGTKLEXK

SEQ ID NO: 448 - protein, 111 aa, Artificial Sequence
  Synthetic peptide
  misc_feature (4)..(4): Xaa can be any naturally occurring amino acid
  misc_feature (82)..(82): Xaa can be any naturally occurring amino acid
  misc_feature (110)..(110): Xaa can be any naturally occurring amino acid
DIVXTQSPDSLAVSLGERATINCRASKSVSTSGYSYIHWYQQKPGQPPKLLIYLASNLESGVPDRFSGSGSGTDFTLTISSXQAEDVAVYYCQHSRELPLTFGQGTKLEXK

SEQ ID NO: 449 - protein, 7 aa, Artificial Sequence
  Synthetic peptide
  MISC_FEATURE (6)..(6): Xaa is T, V, F, or D
SSVSSXY

SEQ ID NO: 450 - protein, 3 aa, Artificial Sequence
  Synthetic peptide
  MISC_FEATURE (1)..(1): Xaa is S, T, Q, or  A
  MISC_FEATURE (3)..(3): Xaa is S, T, D, or Q
XTX

SEQ ID NO: 451 - protein, 9 aa, Artificial Sequence
  Synthetic peptide
  MISC_FEATURE (2)..(2): Xaa is Q, H or S
  MISC_FEATURE (4)..(4): Xaa is H, Y, Q, or S
HXYXRSPLT

SEQ ID NO: 452 - protein, 7 aa, Artificial Sequence
  Synthetic peptide
  MISC_FEATURE (5)..(5): Xaa is T, V, D, or S
YTFTXYT

SEQ ID NO: 453 - protein, 9 aa, Artificial Sequence
  Synthetic peptide
  MISC_FEATURE (2)..(2): Xaa is N, Q, H, D, S, R, or A
AXGDYYVAY

SEQ ID NO: 454 - protein, 9 aa, Artificial Sequence
  Synthetic peptide
  MISC_FEATURE (2)..(2): Xaa is H, Q, S, or T
  MISC_FEATURE (5)..(5): Xaa is T, S, N, or G
QXHYXVPWT

SEQ ID NO: 455 - protein, 7 aa, Artificial Sequence
  Synthetic peptide
  MISC_FEATURE (5)..(5): Xaa is N, S, R, q, s, or a
  MISC_FEATURE (7)..(7): Xaa is w, h, y, or f
FTFSXYX

SEQ ID NO: 456 - protein, 10 aa, Artificial Sequence
  Synthetic peptide
  MISC_FEATURE (5)..(5): Xaa is S, N, A, or T
  MISC_FEATURE (7)..(7): Xaa is Q, S,A, or N
IRLKXDXYAT

SEQ ID NO: 457 - protein, 8 aa, Artificial Sequence
  Synthetic peptide
  MISC_FEATURE (1)..(1): Xaa is N, D, A, or T
  MISC_FEATURE (8)..(8): Xaa is S, T, A, C, Y
XDGPPSGX

SEQ ID NO: 458 - protein, 11 aa, Artificial Sequence
  Synthetic peptide
  MISC_FEATURE (7)..(7): Xaa is D, N, E, Q, S, or A
  MISC_FEATURE (9)..(9): Xaa is Q, S, A, D, or N
QSLVHSXGXTY

SEQ ID NO: 459 - protein, 3 aa, Artificial Sequence
  Synthetic peptide
  MISC_FEATURE (1)..(1): Xaa is K, Q, or R
  MISC_FEATURE (3)..(3): Xaa is S, T, or V
XVX

SEQ ID NO: 460 - protein, 9 aa, Artificial Sequence
  Synthetic peptide
  MISC_FEATURE (2)..(2): Xaa is Q, H, or T
  MISC_FEATURE (3)..(3): Xaa is S, G, T, or D
SXXTHVPYT

SEQ ID NO: 461 - protein, 9 aa, Artificial Sequence
  Synthetic peptide
  MISC_FEATURE (3)..(3): Xaa is F, Y, S, or T
  MISC_FEATURE (5)..(5): Xaa is S, T, Y , or D
YTXTXYTMH

SEQ ID NO: 462 - protein, 8 aa, Artificial Sequence
  Synthetic peptide
  MISC_FEATURE (2)..(2): Xaa is Q, S, A, or N
  MISC_FEATURE (6)..(6): Xaa is T, S, V, D, or G
IXPSSXYT

SEQ ID NO: 463 - protein, 10 aa, Artificial Sequence
  Synthetic peptide
  MISC_FEATURE (1)..(1): Xaa is S, A, T, or V
  MISC_FEATURE (5)..(5): Xaa is L, V, or F
XRGEXGGFAY

SEQ ID NO: 464 - protein, 6 aa, Artificial Sequence
  Synthetic peptide
  MISC_FEATURE (6)..(6): Xaa is W, H, Y, or F
QTIGYX

SEQ ID NO: 465 - protein, 8 aa, Artificial Sequence
  Synthetic peptide
  MISC_FEATURE (3)..(3): Xaa is R or T
  MISC_FEATURE (8)..(8): Xaa is N, Q, S, or A
GYXFTDYX

SEQ ID NO: 466 - protein, 8 aa, Artificial Sequence
  Synthetic peptide
  MISC_FEATURE (2)..(2): Xaa is N, Q, S, or A
  MISC_FEATURE (4)..(4): Xaa is N, Q, S, or A
  MISC_FEATURE (5)..(5): Xaa is N, Q, S, or A
IXPXXGGT

SEQ ID NO: 467 - protein, 8 aa, Artificial Sequence
  Synthetic peptide
  MISC_FEATURE (8)..(8): Xaa is C, Y, S, or A
DYLYFFDX

SEQ ID NO: 468 - protein, 8 aa, Artificial Sequence
  Synthetic peptide
  MISC_FEATURE (4)..(4): Xaa is D, E, S, or A
ISSXSRTI

SEQ ID NO: 469 - protein, 9 aa, Artificial Sequence
  Synthetic peptide
DYGRTYEAY

SEQ ID NO: 470 - protein, 12 aa, Artificial Sequence
  Synthetic peptide
  MISC_FEATURE (8)..(8): Xaa is Q, S, A, D, or N
  MISC_FEATURE (11)..(11): Xaa is Q, S, A, D, or N
QSVLFSSXQKXY

SEQ ID NO: 471 - protein, 3 aa, Artificial Sequence
  Synthetic peptide
  MISC_FEATURE (1)..(1): Xaa is H, Y, F, or W
XAS

SEQ ID NO: 472 - protein, 8 aa, Artificial Sequence
  Synthetic peptide
  MISC_FEATURE (8)..(8): Xaa is N, Q, S, or A
GYSFTFYX

SEQ ID NO: 473 - protein, 8 aa, Artificial Sequence
  Synthetic peptide
  MISC_FEATURE (2)..(2): Xaa is A, S, E, or D
IXPYYGGS

SEQ ID NO: 474 - protein, 12 aa, Artificial Sequence
  Synthetic peptide
ERSGYVFSAMDY

SEQ ID NO: 475 - protein, 8 aa, Artificial Sequence
  Synthetic peptide
  MISC_FEATURE (2)..(2): Xaa is Q, S, A, or N
IXPSSGYT

SEQ ID NO: 476 - protein, 6 aa, Artificial Sequence
  Synthetic peptide
  MISC_FEATURE (2)..(2): Xaa is Q, S, A, D, or N
EXIYSY

SEQ ID NO: 477 - protein, 3 aa, Artificial Sequence
  Synthetic peptide
  MISC_FEATURE (1)..(1): Xaa is Q, S, A, D, or N
XAK

SEQ ID NO: 478 - protein, 116 aa, Artificial Sequence
  Synthetic peptide
  MISC_FEATURE (20)..(20): Xaa is M or V
  MISC_FEATURE (31)..(31): Xaa is T, V, D, or S
  MISC_FEATURE (48)..(48): Xaa is I or M
  MISC_FEATURE (52)..(52): Xaa is Q, S, A, or N
  MISC_FEATURE (70)..(70): Xaa is L or M
  MISC_FEATURE (74)..(74): Xaa is T or K
  MISC_FEATURE (98)..(98): Xaa is N, Q, H, D, S, R,or A
QVQLVQSGAEVKKPGASVKXSCKASGYTFTXYTMHWVRQAPGQGLEWXGFIXPSSGYTDYAQKFQGRVTXTADXSTSTVYMELSSLRSEDTAVYYCAXGDYYVAYWGQGTLVTVSS

SEQ ID NO: 479 - protein, 108 aa, Artificial Sequence
  Synthetic peptide
  MISC_FEATURE (4)..(4): Xaa is L or M
  MISC_FEATURE (21)..(21): Xaa is M or I
  MISC_FEATURE (32)..(32): Xaa is T, V, F, or D
  MISC_FEATURE (48)..(48): Xaa is W or L
  MISC_FEATURE (51)..(51): Xaa is S, t, Q or A
  MISC_FEATURE (53)..(53): Xaa is S,T, D or Q
  MISC_FEATURE (79)..(79): Xaa is M or L
  MISC_FEATURE (84)..(84): Xaa is A or F
  MISC_FEATURE (91)..(91): Xaa is Q, H or S
  MISC_FEATURE (93)..(93): Xaa is H, Y, Q, or S
DIQXTQSPSSLSASVGDRVTXTCTASSSVSSXYFHWYQQKPGKAPKLXIYXTXNLASGVPSRFSGSGSGTDYTLTISSXQPEDXATYYCHXYXRSPLTFGQGTKLEIK

SEQ ID NO: 480 - protein, 117 aa, Artificial Sequence
  Synthetic peptide
  MISC_FEATURE (31)..(31): Xaa is N, S, R, Q or A
  MISC_FEATURE (33)..(33): Xaa is W, H, Y or F
  MISC_FEATURE (55)..(55): Xaa is S, N, A, or T
  MISC_FEATURE (57)..(57): Xaa is Q, S, A, or N
  MISC_FEATURE (99)..(99): Xaa is N, D, or T
  MISC_FEATURE (106)..(106): Xaa is S, T, A, C, or Y
EVQLLESGGGLVQPGGSMRLSCAASGFTFSXYXMNWVRQAPGKGLEWVAQIRLKXDXYATHYADSVKGRFTISRDDSKNTVYLQMNSLRAEDTGVYYCXDGPPSGXWGQGTLLTVSS

SEQ ID NO: 481 - protein, 107 aa, Artificial Sequence
  Synthetic peptide
  MISC_FEATURE (28)..(28): Xaa is Q, S, A, D, or N
  MISC_FEATURE (48)..(48): Xaa is V or I
  MISC_FEATURE (50)..(50): Xaa is S, T, Q or A
  MISC_FEATURE (84)..(84): Xaa is G or A
  MISC_FEATURE (90)..(90): Xaa is H, Q, S or T
  MISC_FEATURE (93)..(93): Xaa is T, S, N, or G
DIQMTQSPSSLSASVGDRVTITCRISEXIYSYLAWYQQKPGKAPKLLXYXAKILVEGVPSRFSGSGSGTDFTLTISSLQPEDFXTYYCQXHYXVPWTFGQGTKLEIK

SEQ ID NO: 482 - protein, 117 aa, Artificial Sequence
  Synthetic peptide
  MISC_FEATURE (20)..(20): Xaa is M or V
  MISC_FEATURE (29)..(29): Xaa is F, Y, S or T
  MISC_FEATURE (31)..(31): Xaa is S, T, Y, or D
  MISC_FEATURE (37)..(37): Xaa is I or V
  MISC_FEATURE (45)..(45): Xaa is Q or L
  MISC_FEATURE (48)..(48): Xaa is I or M
  MISC_FEATURE (52)..(52): Xaa is Q, S, A, or N
  MISC_FEATURE (56)..(56): Xaa is T, S, V, D or G
  MISC_FEATURE (61)..(61): Xaa is I or A
  MISC_FEATURE (62)..(62): Xaa is K or Q
  MISC_FEATURE (65)..(65): Xaa is K or Q
  MISC_FEATURE (66)..(66): Xaa is D or G
  MISC_FEATURE (68)..(68): Xaa is A or V
  MISC_FEATURE (70)..(70): Xaa is L or M
  MISC_FEATURE (74)..(74): Xaa is T or K
  MISC_FEATURE (79)..(79): Xaa is A or V
  MISC_FEATURE (97)..(97): Xaa is S, A, T, or V
  MISC_FEATURE (101)..(97): Xaa is L, V, or F
  misc_feature (101)..(101): Xaa can be any naturally occurring amino acid
QVQLVQSGAEVKKPGASVKXSCKASGYTXTXYTMHWXRQAPGQGXEWXGYIXPSSXYTHYXXKFXXRXTXTADXSTSTXYMELSSLRSEDTAVYYCXRGEXGGFAYWGQGTLVTVSS

SEQ ID NO: 483 - protein, 112 aa, Artificial Sequence
  Synthetic peptide
  MISC_FEATURE (33)..(33): Xaa is D, N, E, Q, S, or A
  MISC_FEATURE (35)..(35): Xaa is Q, S, A, D, or N
  MISC_FEATURE (55)..(55): Xaa is K, Q, or R
  MISC_FEATURE (57)..(57): Xaa is S, T, or V
  MISC_FEATURE (95)..(95): Xaa is Q, H, or T
  MISC_FEATURE (96)..(96): Xaa is S, G, T, or D
DVVMTQSPLSLPVTLGQPASISCRSSQSLVHSDGXTYLNWYQQRPGQSPRLLIYXVXNRFSGVPDRFSGSGSGTDFTLKISRVEAEDVGVYYCSXXTHVPYTFGQGTKLEIK

SEQ ID NO: 484 - protein, 121 aa, Artificial Sequence
  Synthetic peptide
  MISC_FEATURE (20)..(20): Xaa is I or V
  MISC_FEATURE (33)..(33): Xaa is N, Q, S, or A
  MISC_FEATURE (48)..(48): Xaa is I or M
  MISC_FEATURE (52)..(52): Xaa is A, S, E or D
  MISC_FEATURE (68)..(68): Xaa is A or V
  MISC_FEATURE (70)..(70): Xaa is L or M
  MISC_FEATURE (79)..(79): Xaa is A or V
QVQLVQSGAEVKKPGASVKXSCKASGYSFTGYXMNWVRQAPGQGLEWXGNIXPYYGGSTYAQKFQGRXTXTVDTSTSTXYMELSSLRSEDTAVYYCARERSGYVFSAMDYWGQGTLVTVSS

SEQ ID NO: 485 - protein, 112 aa, Artificial Sequence
  Synthetic peptide
  MISC_FEATURE (19)..(19): Xaa is V or A
  MISC_FEATURE (21)..(21): Xaa is M or I
  MISC_FEATURE (34)..(34): Xaa is Q, S, A, D, or N
  MISC_FEATURE (37)..(37): Xaa is Q, S, A, D, or N
  MISC_FEATURE (56)..(56): Xaa is H, Y, F, or W
  MISC_FEATURE (84)..(84): Xaa is V or L
DIVMTQSPDSLAVSLGERXTXNCKSSQSVLFSSXQKXYLAWYQQKPGQPPKLLIYXASTRESGVPDRFSGSGSGTDFTLTISSXQAEDVAVYYCHQYLSSRTFGQGTKLEIK

SEQ ID NO: 486 - protein, 118 aa, Artificial Sequence
  Synthetic peptide
  MISC_FEATURE (54)..(54): Xaa is D, E, S, or A
EVQLVESGGGLVQPGGSLRLSCAASGFTFSSFGMHWVRQAPGKGLEWVAYISSXSRTIYYADSVKGRFTISRDNAKNSLYLQMNSLRAEDTAVYYCARDYGRTYEAYWGQGTLVTVSS

SEQ ID NO: 487 - protein, 111 aa, Artificial Sequence
  Synthetic peptide
  MISC_FEATURE (4)..(4): Xaa is M or L
  MISC_FEATURE (82)..(82): Xaa is V or L
  MISC_FEATURE (110)..(110): Xaa is I or L
DIVXTQSPDSLAVSLGERATINCRASKSVSTSGYSYIHWYQQKPGQPPKLLIYLASNLESGVPDRFSGSGSGTDFTLTISSXQAEDVAVYYCQHSRELPLTFGQGTKLEIK

SEQ ID NO: 488 - protein, 117 aa, Artificial Sequence
  Synthetic peptide
  MISC_FEATURE (28)..(28): Xaa is R or T
  MISC_FEATURE (33)..(33): Xaa is N, Q, S or A
  MISC_FEATURE (52)..(52): Xaa is N, Q, S or A
  MISC_FEATURE (54)..(54): Xaa is N, Q, S or A
  MISC_FEATURE (55)..(55): Xaa is N, Q, S, or A
  MISC_FEATURE (106)..(106): Xaa is C, Y, S, or A
QVQLVQSGAEVKKPGASVKMSCKASGYXFTDYXMHWVRQAPGQGLEWIGYIXPXXGGTNYAQKFQGRATLTVDTSTSTAYMELSSLRSEDTAVYYCARDYLYFFDXWGQGTLLTVSS

SEQ ID NO: 489 - protein, 107 aa, Artificial Sequence
  Synthetic peptide
  MISC_FEATURE (24)..(24): Xaa is L or R
  MISC_FEATURE (32)..(32): Xaa is W, H, Y, or F
DIQMTQSPSSLSASVGDRVTITCLASQTIGTXLAWYQQKPGKAPKLLIYAAASLADGVPSRFSGSGSGTDFTFTISSLQPEDFVTYYCQQLYSIPRTFGQGTKLEIK

SEQ ID NO: 490 - protein, 117 aa, Artificial Sequence
  Synthetic Polypeptide
EVQLLESGGGLVQPGGSMRLSCAASGFTFSNYWMNWVRQAPGKGLEWIAQIRLKSDNYATHYTDSVKGRFTISRDDSKRTVYLQMNSLRAEDTGTYYCSDGPPSGSWGQGTLLTVSS

SEQ ID NO: 491 - protein, 117 aa, Artificial Sequence
  Synthetic Polypeptide
EVQLLESGGGLVQPGGSMRLSCAASGFTFSNYWMNWVRQAPGKGLEWIAQIRLKSDNYATHYADSVKGRFTISRDDSKRTVYLQMNSLRAEDTGTYYCSDGPPSGSWGQGTLLTVSS

SEQ ID NO: 492 - protein, 117 aa, Artificial Sequence
  Synthetic Polypeptide
EVQLLESGGGLVQPGGSMRLSCAASGFTFSNYWMNWVRQAPGKGLEWIAQIRLKSDNYVTHYTDSVKGRFTISRDDSKRTVYLQMNSLRAEDTGIYYCSDGPPSGSWGQGTLLTVSS

SEQ ID NO: 493 - protein, 117 aa, Artificial Sequence
  Synthetic Polypeptide
EVQLLESGGGLVQPGGSMRLSCAASGFTFSNYWMNWVRQAPGKGLEWIAQIRLKSDNYATHYTDSVKGRFTISRDDSKSTVYLQMNSLRAEDTGTYYCNDGPPSGSWGQGTLLTVSS

SEQ ID NO: 494 - protein, 117 aa, Artificial Sequence
  Synthetic Polypeptide
EVQLLESGGGLVQPGGSMRLSCAASGFTFSNYWMNWVRQAPGKGLEWLAQIRLKSDNYATHYTDSVKGRFTISRDDSKRTVYLQMNSLRAEDTGIYYCSDGPPSGSWGQGTLLTVSS

SEQ ID NO: 495 - protein, 117 aa, Artificial Sequence
  Synthetic Polypeptide
EVQLLESGGGLVQPGGSMRLSCAASGFTFSNYWMNWVRQAPGKGLEWLAQIRLKSDNYVTHYADSVKGRFTISRDDSKRTVYLQMNSLRAEDTGTYYCNDGPPSGSWGQGTLLTVSS

SEQ ID NO: 496 - protein, 116 aa, Artificial Sequence
  Synthetic Polypeptide
QVQLVQSGAEVKKPGASVKMSCKASGYTFTTYTIHWVRQAPGQGLEWIGFINPSSGYTEYAQKFQGRVTLTADKSTSTVYMELSSLRSEDTAVYFCANGDYYVAYWGQGTLVTVSS

SEQ ID NO: 497 - protein, 116 aa, Artificial Sequence
  Synthetic Polypeptide
QVQLVQSGAEVKKPGASVKMSCKASGYTFTTYTMHWVRQAPGQGLEWIGVINPSSGYTEYAQKFQGRVTLTADKSTSTVYMELSSLRSEDTAVYFCANGDYYVGYWGQGTLVTVSS

SEQ ID NO: 498 - protein, 116 aa, Artificial Sequence
  Synthetic Polypeptide
QVQLVQSGAEVKKPGASVKMSCKASGYTFTTYTIHWVRQAPGQGLEWIGVINPSSGYTDYAQKFQGRVTLTADKSTSTVYMELSSLRSEDTAVYFCANGDYYVGYWGQGTLVTVSS

SEQ ID NO: 499 - protein, 116 aa, Artificial Sequence
  Synthetic Polypeptide
QVQLVQSGAEVKKPGASVKMSCKASGYTFTTYTMHWVRQAPGQGLEWIGFINPSSGYTEYAQKFQGRVTLTADKSTSTVYMELSSLRSEDTAVYYCANGDYYVGYWGQGTLVTVSS

SEQ ID NO: 500 - protein, 116 aa, Artificial Sequence
  Synthetic Polypeptide
QVQLVQSGAEVKKPGASVKMSCKASGYTFTTYTIHWVRQAPGQGLEWIGVINPSSGYTEYAQKFQGRVTLTADKSTSTVYMELSSLRSEDTAVYFCANGDYYVAYWGQGTLVTVSS

SEQ ID NO: 501 - protein, 116 aa, Artificial Sequence
  Synthetic Polypeptide
QVQLVQSGAEVKKPGASVKMSCKASGYTFTTYTMHWVRQAPGQGLEWIGFINPSSGYTEYAQKFQGRVTLTADKSTSTVYMELSSLRSEDTAVYFCANGDYYVGYWGQGTLVTVSS

SEQ ID NO: 502 - protein, 117 aa, Artificial Sequence
  Synthetic Polypeptide
  MISC_FEATURE (48)..(48): Xaa is any aliphatic amino acid, optionally Ile or Leu
  MISC_FEATURE (59)..(59): Xaa is any aliphatic amino acid, optionally, Ala or Val
  MISC_FEATURE (63)..(63): Xaa is any aliphatic or any amino acid with a polar side chain, optionally, Ala or Thr
  MISC_FEATURE (79)..(79): Xaa is any basic amino acid or any amino acid with a polar side chain, optionally Arg or Ser
  MISC_FEATURE (95)..(95): Xaa is any aliphatic amino acid or any amino acid with a polar side chain, optionally, Thr or Ile
  MISC_FEATURE (99)..(99): Xaa is any acidic amino acid or any amino acid with a polar side chain, optionally, Ser or Asn
EVQLLESGGGLVQPGGSMRLSCAASGFTFSNYWMNWVRQAPGKGLEWXAQIRLKSDNYXTHYXDSVKGRFTISRDDSKXTVYLQMNSLRAEDTGXYYCXDGPPSGSWGQGTLLTVSS

SEQ ID NO: 503 - protein, 116 aa, Artificial Sequence
  Synthetic Polypeptide
  MISC_FEATURE (34)..(34): Xaa is any aliphatic amino acid or any amino acid comprising a sulfur containing side chain; optionally, Ile or Met
  MISC_FEATURE (50)..(50): Xaa is any aliphatic amino acid or any aromatic amino acid, optionally, Phe or Val
  MISC_FEATURE (59)..(59): Xaa is any acidic amino acid, optionally, Glu or Asp
  MISC_FEATURE (95)..(95): Xaa is any aromatic amino acid, optionally, Phe or Tyr
  MISC_FEATURE (104)..(104): Xaa is any aliphatic amino acid, optionally, Gly or Ala
QVQLVQSGAEVKKPGASVKMSCKASGYTFTTYTXHWVRQAPGQGLEWIGXINPSSGYTXYAQKFQGRVTLTADKSTSTVYMELSSLRSEDTAVYXCANGDYYVXYWGQGTLVTVSS

SEQ ID NO: 504 - protein, 8 aa, Artificial Sequence
  Synthetic Polypeptide
GYTFTTYT

SEQ ID NO: 505 - protein, 8 aa, Artificial Sequence
  Synthetic Polypeptide
INPSSGYT

SEQ ID NO: 506 - protein, 9 aa, Artificial Sequence
  Synthetic Polypeptide
  MISC_FEATURE (8)..(8): Xaa is any aliphatic amino acid, optionally, Gly or Ala
ANGDYYVXY

SEQ ID NO: 507 - protein, 8 aa, Artificial Sequence
  Synthetic Polypeptide
GFTFSNYW

SEQ ID NO: 508 - protein, 10 aa, Artificial Sequence
  Synthetic Polypeptide
  MISC_FEATURE (9)..(9): Xaa is any aliphatic amino acid, optionally, Ala or Val
IRLKSDNYXT

SEQ ID NO: 509 - protein, 8 aa, Artificial Sequence
  Synthetic Polypeptide
  MISC_FEATURE (1)..(1): Xaa is any acidic amino acid or any amino acid with a polar side chain, optionally, Ser or Asn
XDGPPSGS

SEQ ID NO: 510 - protein, 117 aa, Artificial Sequence
  Synthetic Polypeptide
EVKLEESGGGLVQPGGSMKLSCVASGFTFSNYWMNWVRQSPEKGLEWVAQIRLKSDNYATHYAESVKGRFTISRDDSKSSVYLQMNNLRAEDTGIYYCNDGPPSGCWGQGTTLTVSS

SEQ ID NO: 511 - protein, 107 aa, Artificial Sequence
  Synthetic Polypeptide
DIQMTQSPASLSASVGETVTITCRASENIYSYLAWYQQKQGKSPQLLVYNAKILVEGVPSRFSGSGSGTQFSLKINSLQPEDFGNYYCQHHYTVPWTFGGGTKLEIK

SEQ ID NO: 512 - protein, 108 aa, Artificial Sequence
  Synthetic Polypeptide
QIVLTQSPAIMSASLGERVTMTCTASSSVSSSYLHWYQQKPGSSPKLWIYSTSNLASGVPARFSGSGSGTSYSLTISSMEAEDAATYYCHQYHRSPLTFGAGTKLELK

SEQ ID NO: 513 - protein, 116 aa, Artificial Sequence
  Synthetic Polypeptide
QVQLQQSAAELARPGASVKMSCKASGYTFTSYTMHWVKQRPGQGLEWIGFINPSSGYTDYNQKFKDKTTLTADKSSSTAYMQLSSLTSEDSAVYYCANGDYYVAYWGQGTLVTVSA